European Patent Specification EP 3 636 277 B1, published July 2, 2025. Title: PEPTIDES, DEVICES, AND METHODS FOR THE DETECTION OF ANAPLASMA ANTIBODIES. Applicant: Abaxis, Inc. Mehra, Rajesh K. Aron, Kenneth P. Bleile, Dennis M. Walker, Jeremy D. Rogers, Andrews P. Forsyth, Timothy P. Cuesico, Chistina R. The sequence listing filed with the application follows.

SEQUENCE LISTING (543 sequences)

SEQ ID NO: 1 - protein, 36 aa, Artificial Sequence
  Anaplasma antigenic peptide
  MISC_FEATURE (9)..(9): Xaa is Ile, Pro or His
  MISC_FEATURE (17)..(17): Xaa is Ile, Trp or Tyr
  MISC_FEATURE (21)..(21): Xaa is Arg, Asp or Asn
  MISC_FEATURE (28)..(28): Xaa is Glu or Asn
  MISC_FEATURE (31)..(31): Xaa is Leu of Val
ETRVAYPYXKDGRTVKXDSHXFDWQTPXPKXGFKDC

SEQ ID NO: 2 - protein, 21 aa, Artificial Sequence
  Anaplasma antigenic peptide
  MISC_FEATURE (3)..(3): Xaa is Leu, Val or Ala
  MISC_FEATURE (7)..(7): Xaa is Lys, Asn or Gln
  MISC_FEATURE (11)..(11): Xaa is Arg, Asp or Asn
  MISC_FEATURE (15)..(15): Xaa is Glu, Asn or Gln
IEXGYEXFKTXGIRXSGTKEC

SEQ ID NO: 3 - protein, 67 aa, Artificial Sequence
  Anaplasma antigenic peptide
  MISC_FEATURE (5)..(5): Xaa is Val or Ala
  MISC_FEATURE (7)..(7): Xaa is Gly, Ile or His
  MISC_FEATURE (11)..(11): Xaa is Glu, Asn or Gln
  MISC_FEATURE (18)..(18): Xaa is Asp or Asn
  MISC_FEATURE (21)..(21): Xaa is Arg, Asp or Asn
  MISC_FEATURE (25)..(25): Xaa is Gln, Asp or Glu
  MISC_FEATURE (28)..(28): Xaa is Glu or Asn
  MISC_FEATURE (31)..(31): Xaa is Leu or Val
  MISC_FEATURE (45)..(45): Xaa is Lys or Gln
  MISC_FEATURE (48)..(48): Xaa is Phe or Val
  MISC_FEATURE (51)..(51): Xaa is Asp or Asn
  MISC_FEATURE (54)..(54): Xaa is Glu or Gln
  MISC_FEATURE (57)..(57): Xaa is Ser or Gln
  MISC_FEATURE (60)..(60): Xaa is Phe or Trp
  MISC_FEATURE (63)..(63): Xaa is Ile or Val
  MISC_FEATURE (66)..(66): Xaa is Gln or Asp
ETKVXYXYLKXGRTVKLXSHXFDWXTPXPKXGFKDGGGGGKDGTXVEXKAXKFXWNXPDXRIXFKXC

SEQ ID NO: 4 - protein, 27 aa, Artificial Sequence
  Anaplasma antigenic peptide
  MISC_FEATURE (6)..(6): Xaa is Lys or Gln
  MISC_FEATURE (9)..(9): Xaa is Phe or Val
  MISC_FEATURE (12)..(12): Xaa is Asp or Asn
  MISC_FEATURE (15)..(15): Xaa is Glu or Gln
  MISC_FEATURE (18)..(18): Xaa is Ser or Gln
  MISC_FEATURE (21)..(21): Xaa is Phe or Trp
  MISC_FEATURE (24)..(24): Xaa is Ile or Val
  MISC_FEATURE (27)..(27): Xaa is Gln or Asp
CKDGTXVEXKAXKFXWNXPDXRIXFKX

SEQ ID NO: 5 - protein, 40 aa, Artificial Sequence
  Anaplasma antigenic peptide
  MISC_FEATURE (2)..(2): Xaa is Ile or Val
  MISC_FEATURE (10)..(10): Xaa is Ser or Tyr
  MISC_FEATURE (23)..(23): Xaa is Glu or Asn
CXGGKSPARXTEERVAGDLDHKXVDSDKKHDAEKTEEKRH

SEQ ID NO: 6 - protein, 31 aa, Artificial Sequence
  Anaplasma antigenic peptide
CGKILNLVSAVQEKKPPEAPAADEAAGPATH

SEQ ID NO: 7 - protein, 27 aa, Artificial Sequence
  Anaplasma antigenic peptide
  MISC_FEATURE (5)..(5): Xaa is Ser or Gln
  MISC_FEATURE (9)..(9): Xaa is Phe or Tyr
  MISC_FEATURE (13)..(13): Xaa is Arg or His
  MISC_FEATURE (16)..(16): Xaa is Trp or Tyr
  MISC_FEATURE (18)..(18): Xaa is Ser or Gln
  MISC_FEATURE (22)..(22): Xaa is Lys or His
  MISC_FEATURE (27)..(27): Xaa is Asn or Asp
CKDGXRVEXKAEXFNXQXPNPXIKYRX

SEQ ID NO: 8 - protein, 31 aa, Artificial Sequence
  Anaplasma antigenic peptide
  MISC_FEATURE (10)..(10): Xaa is Val, Leu or Ile
  MISC_FEATURE (11)..(11): Xaa is Ala or Leu
CGKILNLVSXXNEKKPPEAPAADEAAGPATH

SEQ ID NO: 9 - protein, 36 aa, Artificial Sequence
  Anaplasma antigenic peptide
  MISC_FEATURE (5)..(5): Xaa is Val or Ala
  MISC_FEATURE (7)..(7): Xaa is Gly, Ile or His
  MISC_FEATURE (11)..(11): Xaa is Glu, Asn or Gln
  MISC_FEATURE (21)..(21): Xaa is Arg, Asp or Asn
  MISC_FEATURE (25)..(25): Xaa is Gln, Asp or Glu
  MISC_FEATURE (28)..(28): Xaa is Glu or Asn
  MISC_FEATURE (31)..(31): Xaa is Leu or Val
ETKVXYXYLKXGRTVKLDSHXFDWXTPXPKXGFKDC

SEQ ID NO: 10 - protein, 36 aa, Artificial Sequence
  Anaplasma antigenic peptide
ETRVAYPYIKDGRTVKIDSHRFDWQTPEPKLGFKDC

SEQ ID NO: 11 - protein, 36 aa, Artificial Sequence
  Anaplasma antigenic peptide
ETRVAYPYPKDGRTVKIDSHRFDWQTPEPKLGFKDC

SEQ ID NO: 12 - protein, 36 aa, Artificial Sequence
  Anaplasma antigenic peptide
ETRVAYPYHKDGRTVKIDSHRFDWQTPEPKLGFKDC

SEQ ID NO: 13 - protein, 36 aa, Artificial Sequence
  Anaplasma antigenic peptide
ETRVAYPYIKDGRTVKWDSHRFDWQTPEPKLGFKDC

SEQ ID NO: 14 - protein, 36 aa, Artificial Sequence
  Anaplasma antigenic peptide
ETRVAYPYIKDGRTVKYDSHRFDWQTPEPKLGFKDC

SEQ ID NO: 15 - protein, 36 aa, Artificial Sequence
  Anaplasma antigenic peptide
ETRVAYPYPKDGRTVKWDSHRFDWQTPEPKLGFKDC

SEQ ID NO: 16 - protein, 36 aa, Artificial Sequence
  Anaplasma antigenic peptide
ETRVAYPYPKDGRTVKYDSHRFDWQTPEPKLGFKDC

SEQ ID NO: 17 - protein, 36 aa, Artificial Sequence
  Anaplasma antigenic peptide
ETRVAYPYHKDGRTVKWDSHRFDWQTPEPKLGFKDC

SEQ ID NO: 18 - protein, 36 aa, Artificial Sequence
  Anaplasma antigenic peptide
ETRVAYPYHKDGRTVKYDSHRFDWQTPEPKLGFKDC

SEQ ID NO: 19 - protein, 36 aa, Artificial Sequence
  Anaplasma antigenic peptide
ETRVAYPYIKDGRTVKIDSHDFDWQTPEPKLGFKDC

SEQ ID NO: 20 - protein, 36 aa, Artificial Sequence
  Anaplasma antigenic peptide
ETRVAYPYIKDGRTVKWDSHDFDWQTPEPKLGFKDC

SEQ ID NO: 21 - protein, 36 aa, Artificial Sequence
  Anaplasma antigenic peptide
ETRVAYPYIKDGRTVKYDSHDFDWQTPEPKLGFKDC

SEQ ID NO: 22 - protein, 36 aa, Artificial Sequence
  Anaplasma antigenic peptide
ETRVAYPYPKDGRTVKIDSHDFDWQTPEPKLGFKDC

SEQ ID NO: 23 - protein, 36 aa, Artificial Sequence
  Anaplasma antigenic peptide
ETRVAYPYPKDGRTVKWDSHDFDWQTPEPKLGFKDC

SEQ ID NO: 24 - protein, 36 aa, Artificial Sequence
  Anaplasma antigenic peptide
ETRVAYPYPKDGRTVKYDSHDFDWQTPEPKLGFKDC

SEQ ID NO: 25 - protein, 36 aa, Artificial Sequence
  Anaplasma antigenic peptide
ETRVAYPYHKDGRTVKIDSHDFDWQTPEPKLGFKDC

SEQ ID NO: 26 - protein, 36 aa, Artificial Sequence
  Anaplasma antigenic peptide
ETRVAYPYHKDGRTVKWDSHDFDWQTPEPKLGFKDC

SEQ ID NO: 27 - protein, 36 aa, Artificial Sequence
  Anaplasma antigenic peptide
ETRVAYPYHKDGRTVKYDSHDFDWQTPEPKLGFKDC

SEQ ID NO: 28 - protein, 36 aa, Artificial Sequence
  Anaplasma antigenic peptide
ETRVAYPYIKDGRTVKIDSHNFDWQTPEPKLGFKDC

SEQ ID NO: 29 - protein, 36 aa, Artificial Sequence
  Anaplasma antigenic peptide
ETRVAYPYIKDGRTVKWDSHNFDWQTPEPKLGFKDC

SEQ ID NO: 30 - protein, 36 aa, Artificial Sequence
  Anaplasma antigenic peptide
ETRVAYPYIKDGRTVKYDSHNFDWQTPEPKLGFKDC

SEQ ID NO: 31 - protein, 36 aa, Artificial Sequence
  Anaplasma antigenic peptide
ETRVAYPYPKDGRTVKIDSHNFDWQTPEPKLGFKDC

SEQ ID NO: 32 - protein, 36 aa, Artificial Sequence
  Anaplasma antigenic peptide
ETRVAYPYPKDGRTVKWDSHNFDWQTPEPKLGFKDC

SEQ ID NO: 33 - protein, 36 aa, Artificial Sequence
  Anaplasma antigenic peptide
ETRVAYPYPKDGRTVKYDSHNFDWQTPEPKLGFKDC

SEQ ID NO: 34 - protein, 36 aa, Artificial Sequence
  Anaplasma antigenic peptide
ETRVAYPYHKDGRTVKIDSHNFDWQTPEPKLGFKDC

SEQ ID NO: 35 - protein, 36 aa, Artificial Sequence
  Anaplasma antigenic peptide
ETRVAYPYHKDGRTVKWDSHNFDWQTPEPKLGFKDC

SEQ ID NO: 36 - protein, 36 aa, Artificial Sequence
  Anaplasma antigenic peptide
ETRVAYPYHKDGRTVKYDSHNFDWQTPEPKLGFKDC

SEQ ID NO: 37 - protein, 36 aa, Artificial Sequence
  Anaplasma antigenic peptide
ETRVAYPYIKDGRTVKIDSHRFDWQTPNPKLGFKDC

SEQ ID NO: 38 - protein, 36 aa, Artificial Sequence
  Anaplasma antigenic peptide
ETRVAYPYPKDGRTVKIDSHRFDWQTPNPKLGFKDC

SEQ ID NO: 39 - protein, 36 aa, Artificial Sequence
  Anaplasma antigenic peptide
ETRVAYPYHKDGRTVKIDSHRFDWQTPNPKLGFKDC

SEQ ID NO: 40 - protein, 36 aa, Artificial Sequence
  Anaplasma antigenic peptide
ETRVAYPYIKDGRTVKWDSHRFDWQTPNPKLGFKDC

SEQ ID NO: 41 - protein, 36 aa, Artificial Sequence
  Anaplasma antigenic peptide
ETRVAYPYIKDGRTVKYDSHRFDWQTPNPKLGFKDC

SEQ ID NO: 42 - protein, 36 aa, Artificial Sequence
  Anaplasma antigenic peptide
ETRVAYPYPKDGRTVKWDSHRFDWQTPNPKLGFKDC

SEQ ID NO: 43 - protein, 36 aa, Artificial Sequence
  Anaplasma antigenic peptide
ETRVAYPYPKDGRTVKYDSHRFDWQTPNPKLGFKDC

SEQ ID NO: 44 - protein, 36 aa, Artificial Sequence
  Anaplasma antigenic peptide
ETRVAYPYHKDGRTVKWDSHRFDWQTPNPKLGFKDC

SEQ ID NO: 45 - protein, 36 aa, Artificial Sequence
  Anaplasma antigenic peptide
ETRVAYPYHKDGRTVKYDSHRFDWQTPNPKLGFKDC

SEQ ID NO: 46 - protein, 36 aa, Artificial Sequence
  Anaplasma antigenic peptide
ETRVAYPYIKDGRTVKIDSHDFDWQTPNPKLGFKDC

SEQ ID NO: 47 - protein, 36 aa, Artificial Sequence
  Anaplasma antigenic peptide
ETRVAYPYIKDGRTVKWDSHDFDWQTPNPKLGFKDC

SEQ ID NO: 48 - protein, 36 aa, Artificial Sequence
  Anaplasma antigenic peptide
ETRVAYPYIKDGRTVKYDSHDFDWQTPNPKLGFKDC

SEQ ID NO: 49 - protein, 36 aa, Artificial Sequence
  Anaplasma antigenic peptide
ETRVAYPYPKDGRTVKIDSHDFDWQTPNPKLGFKDC

SEQ ID NO: 50 - protein, 36 aa, Artificial Sequence
  Anaplasma antigenic peptide
ETRVAYPYPKDGRTVKWDSHDFDWQTPNPKLGFKDC

SEQ ID NO: 51 - protein, 36 aa, Artificial Sequence
  Anaplasma antigenic peptide
ETRVAYPYPKDGRTVKYDSHDFDWQTPNPKLGFKDC

SEQ ID NO: 52 - protein, 36 aa, Artificial Sequence
  Anaplasma antigenic peptide
ETRVAYPYHKDGRTVKIDSHDFDWQTPNPKLGFKDC

SEQ ID NO: 53 - protein, 36 aa, Artificial Sequence
  Anaplasma antigenic peptide
ETRVAYPYHKDGRTVKWDSHDFDWQTPNPKLGFKDC

SEQ ID NO: 54 - protein, 36 aa, Artificial Sequence
  Anaplasma antigenic peptide
ETRVAYPYHKDGRTVKYDSHDFDWQTPNPKLGFKDC

SEQ ID NO: 55 - protein, 36 aa, Artificial Sequence
  Anaplasma antigenic peptide
ETRVAYPYIKDGRTVKIDSHNFDWQTPNPKLGFKDC

SEQ ID NO: 56 - protein, 36 aa, Artificial Sequence
  Anaplasma antigenic peptide
ETRVAYPYIKDGRTVKWDSHNFDWQTPNPKLGFKDC

SEQ ID NO: 57 - protein, 36 aa, Artificial Sequence
  Anaplasma antigenic peptide
ETRVAYPYIKDGRTVKYDSHNFDWQTPNPKLGFKDC

SEQ ID NO: 58 - protein, 36 aa, Artificial Sequence
  Anaplasma antigenic peptide
ETRVAYPYPKDGRTVKIDSHNFDWQTPNPKLGFKDC

SEQ ID NO: 59 - protein, 36 aa, Artificial Sequence
  Anaplasma antigenic peptide
ETRVAYPYPKDGRTVKWDSHNFDWQTPNPKLGFKDC

SEQ ID NO: 60 - protein, 36 aa, Artificial Sequence
  Anaplasma antigenic peptide
ETRVAYPYPKDGRTVKYDSHNFDWQTPNPKLGFKDC

SEQ ID NO: 61 - protein, 36 aa, Artificial Sequence
  Anaplasma antigenic peptide
ETRVAYPYHKDGRTVKIDSHNFDWQTPNPKLGFKDC

SEQ ID NO: 62 - protein, 36 aa, Artificial Sequence
  Anaplasma antigenic peptide
ETRVAYPYHKDGRTVKWDSHNFDWQTPNPKLGFKDC

SEQ ID NO: 63 - protein, 36 aa, Artificial Sequence
  Anaplasma antigenic peptide
ETRVAYPYHKDGRTVKYDSHNFDWQTPNPKLGFKDC

SEQ ID NO: 64 - protein, 36 aa, Artificial Sequence
  Anaplasma antigenic peptide
ETRVAYPYIKDGRTVKIDSHRFDWQTPEPKVGFKDC

SEQ ID NO: 65 - protein, 36 aa, Artificial Sequence
  Anaplasma antigenic peptide
ETRVAYPYPKDGRTVKIDSHRFDWQTPEPKVGFKDC

SEQ ID NO: 66 - protein, 36 aa, Artificial Sequence
  Anaplasma antigenic peptide
ETRVAYPYHKDGRTVKIDSHRFDWQTPEPKVGFKDC

SEQ ID NO: 67 - protein, 36 aa, Artificial Sequence
  Anaplasma antigenic peptide
ETRVAYPYIKDGRTVKWDSHRFDWQTPEPKVGFKDC

SEQ ID NO: 68 - protein, 36 aa, Artificial Sequence
  Anaplasma antigenic peptide
ETRVAYPYIKDGRTVKYDSHRFDWQTPEPKVGFKDC

SEQ ID NO: 69 - protein, 36 aa, Artificial Sequence
  Anaplasma antigenic peptide
ETRVAYPYPKDGRTVKWDSHRFDWQTPEPKVGFKDC

SEQ ID NO: 70 - protein, 36 aa, Artificial Sequence
  Anaplasma antigenic peptide
ETRVAYPYPKDGRTVKYDSHRFDWQTPEPKVGFKDC

SEQ ID NO: 71 - protein, 36 aa, Artificial Sequence
  Anaplasma antigenic peptide
ETRVAYPYHKDGRTVKWDSHRFDWQTPEPKVGFKDC

SEQ ID NO: 72 - protein, 36 aa, Artificial Sequence
  Anaplasma antigenic peptide
ETRVAYPYHKDGRTVKYDSHRFDWQTPEPKVGFKDC

SEQ ID NO: 73 - protein, 36 aa, Artificial Sequence
  Anaplasma antigenic peptide
ETRVAYPYIKDGRTVKIDSHDFDWQTPEPKVGFKDC

SEQ ID NO: 74 - protein, 36 aa, Artificial Sequence
  Anaplasma antigenic peptide
ETRVAYPYIKDGRTVKWDSHDFDWQTPEPKVGFKDC

SEQ ID NO: 75 - protein, 36 aa, Artificial Sequence
  Anaplasma antigenic peptide
ETRVAYPYIKDGRTVKYDSHDFDWQTPEPKVGFKDC

SEQ ID NO: 76 - protein, 36 aa, Artificial Sequence
  Anaplasma antigenic peptide
ETRVAYPYPKDGRTVKIDSHDFDWQTPEPKVGFKDC

SEQ ID NO: 77 - protein, 36 aa, Artificial Sequence
  Anaplasma antigenic peptide
ETRVAYPYPKDGRTVKWDSHDFDWQTPEPKVGFKDC

SEQ ID NO: 78 - protein, 36 aa, Artificial Sequence
  Anaplasma antigenic peptide
ETRVAYPYPKDGRTVKYDSHDFDWQTPEPKVGFKDC

SEQ ID NO: 79 - protein, 36 aa, Artificial Sequence
  Anaplasma antigenic peptide
ETRVAYPYHKDGRTVKIDSHDFDWQTPEPKVGFKDC

SEQ ID NO: 80 - protein, 36 aa, Artificial Sequence
  Anaplasma antigenic peptide
ETRVAYPYHKDGRTVKWDSHDFDWQTPEPKVGFKDC

SEQ ID NO: 81 - protein, 36 aa, Artificial Sequence
  Anaplasma antigenic peptide
ETRVAYPYHKDGRTVKYDSHDFDWQTPEPKVGFKDC

SEQ ID NO: 82 - protein, 36 aa, Artificial Sequence
  Anaplasma antigenic peptide
ETRVAYPYIKDGRTVKIDSHNFDWQTPEPKVGFKDC

SEQ ID NO: 83 - protein, 36 aa, Artificial Sequence
  Anaplasma antigenic peptide
ETRVAYPYIKDGRTVKWDSHNFDWQTPEPKVGFKDC

SEQ ID NO: 84 - protein, 36 aa, Artificial Sequence
  Anaplasma antigenic peptide
ETRVAYPYIKDGRTVKYDSHNFDWQTPEPKVGFKDC

SEQ ID NO: 85 - protein, 36 aa, Artificial Sequence
  Anaplasma antigenic peptide
ETRVAYPYPKDGRTVKIDSHNFDWQTPEPKVGFKDC

SEQ ID NO: 86 - protein, 36 aa, Artificial Sequence
  Anaplasma antigenic peptide
ETRVAYPYPKDGRTVKWDSHNFDWQTPEPKVGFKDC

SEQ ID NO: 87 - protein, 36 aa, Artificial Sequence
  Anaplasma antigenic peptide
ETRVAYPYPKDGRTVKYDSHNFDWQTPEPKVGFKDC

SEQ ID NO: 88 - protein, 36 aa, Artificial Sequence
  Anaplasma antigenic peptide
ETRVAYPYHKDGRTVKIDSHNFDWQTPEPKVGFKDC

SEQ ID NO: 89 - protein, 36 aa, Artificial Sequence
  Anaplasma antigenic peptide
ETRVAYPYHKDGRTVKWDSHNFDWQTPEPKVGFKDC

SEQ ID NO: 90 - protein, 36 aa, Artificial Sequence
  Anaplasma antigenic peptide
ETRVAYPYHKDGRTVKYDSHNFDWQTPEPKVGFKDC

SEQ ID NO: 91 - protein, 36 aa, Artificial Sequence; identical to SEQ ID NO: 37
  Anaplasma antigenic peptide

SEQ ID NO: 92 - protein, 36 aa, Artificial Sequence; identical to SEQ ID NO: 38
  Anaplasma antigenic peptide

SEQ ID NO: 93 - protein, 36 aa, Artificial Sequence; identical to SEQ ID NO: 39
  Anaplasma antigenic peptide

SEQ ID NO: 94 - protein, 36 aa, Artificial Sequence; identical to SEQ ID NO: 40
  Anaplasma antigenic peptide

SEQ ID NO: 95 - protein, 36 aa, Artificial Sequence; identical to SEQ ID NO: 41
  Anaplasma antigenic peptide

SEQ ID NO: 96 - protein, 36 aa, Artificial Sequence; identical to SEQ ID NO: 42
  Anaplasma antigenic peptide

SEQ ID NO: 97 - protein, 36 aa, Artificial Sequence; identical to SEQ ID NO: 43
  Anaplasma antigenic peptide

SEQ ID NO: 98 - protein, 36 aa, Artificial Sequence; identical to SEQ ID NO: 44
  Anaplasma antigenic peptide

SEQ ID NO: 99 - protein, 36 aa, Artificial Sequence; identical to SEQ ID NO: 45
  Anaplasma antigenic peptide

SEQ ID NO: 100 - protein, 36 aa, Artificial Sequence; identical to SEQ ID NO: 46
  Anaplasma antigenic peptide

SEQ ID NO: 101 - protein, 36 aa, Artificial Sequence; identical to SEQ ID NO: 47
  Anaplasma antigenic peptide

SEQ ID NO: 102 - protein, 36 aa, Artificial Sequence; identical to SEQ ID NO: 48
  Anaplasma antigenic peptide

SEQ ID NO: 103 - protein, 36 aa, Artificial Sequence; identical to SEQ ID NO: 49
  Anaplasma antigenic peptide

SEQ ID NO: 104 - protein, 36 aa, Artificial Sequence; identical to SEQ ID NO: 50
  Anaplasma antigenic peptide

SEQ ID NO: 105 - protein, 36 aa, Artificial Sequence; identical to SEQ ID NO: 51
  Anaplasma antigenic peptide

SEQ ID NO: 106 - protein, 36 aa, Artificial Sequence; identical to SEQ ID NO: 52
  Anaplasma antigenic peptide

SEQ ID NO: 107 - protein, 36 aa, Artificial Sequence; identical to SEQ ID NO: 53
  Anaplasma antigenic peptide

SEQ ID NO: 108 - protein, 36 aa, Artificial Sequence; identical to SEQ ID NO: 54
  Anaplasma antigenic peptide

SEQ ID NO: 109 - protein, 36 aa, Artificial Sequence; identical to SEQ ID NO: 55
  Anaplasma antigenic peptide

SEQ ID NO: 110 - protein, 36 aa, Artificial Sequence; identical to SEQ ID NO: 56
  Anaplasma antigenic peptide

SEQ ID NO: 111 - protein, 36 aa, Artificial Sequence; identical to SEQ ID NO: 57
  Anaplasma antigenic peptide

SEQ ID NO: 112 - protein, 36 aa, Artificial Sequence; identical to SEQ ID NO: 58
  Anaplasma antigenic peptide

SEQ ID NO: 113 - protein, 36 aa, Artificial Sequence; identical to SEQ ID NO: 59
  Anaplasma antigenic peptide

SEQ ID NO: 114 - protein, 36 aa, Artificial Sequence; identical to SEQ ID NO: 60
  Anaplasma antigenic peptide

SEQ ID NO: 115 - protein, 36 aa, Artificial Sequence; identical to SEQ ID NO: 61
  Anaplasma antigenic peptide

SEQ ID NO: 116 - protein, 36 aa, Artificial Sequence; identical to SEQ ID NO: 62
  Anaplasma antigenic peptide

SEQ ID NO: 117 - protein, 36 aa, Artificial Sequence; identical to SEQ ID NO: 63
  Anaplasma antigenic peptide

SEQ ID NO: 118 - protein, 21 aa, Artificial Sequence
  Anaplasma antigenic peptide
IELGYEKFKTRGIRESGTKEC

SEQ ID NO: 119 - protein, 21 aa, Artificial Sequence
  Anaplasma antigenic peptide
IELGYENFKTRGIRESGTKEC

SEQ ID NO: 120 - protein, 21 aa, Artificial Sequence
  Anaplasma antigenic peptide
IELGYEQFKTRGIRESGTKEC

SEQ ID NO: 121 - protein, 21 aa, Artificial Sequence
  Anaplasma antigenic peptide
IEVGYEKFKTRGIRESGTKEC

SEQ ID NO: 122 - protein, 21 aa, Artificial Sequence
  Anaplasma antigenic peptide
IEAGYEKFKTRGIRESGTKEC

SEQ ID NO: 123 - protein, 21 aa, Artificial Sequence
  Anaplasma antigenic peptide
IEVGYENFKTRGIRESGTKEC

SEQ ID NO: 124 - protein, 21 aa, Artificial Sequence
  Anaplasma antigenic peptide
IEVGYEQFKTRGIRESGTKEC

SEQ ID NO: 125 - protein, 21 aa, Artificial Sequence
  Anaplasma antigenic peptide
IEAGYENFKTRGIRESGTKEC

SEQ ID NO: 126 - protein, 21 aa, Artificial Sequence
  Anaplasma antigenic peptide
IEAGYEQFKTRGIRESGTKEC

SEQ ID NO: 127 - protein, 21 aa, Artificial Sequence
  Anaplasma antigenic peptide
IELGYEKFKTDGIRESGTKEC

SEQ ID NO: 128 - protein, 21 aa, Artificial Sequence
  Anaplasma antigenic peptide
IELGYENFKTDGIRESGTKEC

SEQ ID NO: 129 - protein, 21 aa, Artificial Sequence
  Anaplasma antigenic peptide
IELGYEQFKTDGIRESGTKEC

SEQ ID NO: 130 - protein, 21 aa, Artificial Sequence
  Anaplasma antigenic peptide
IEVGYEKFKTDGIRESGTKEC

SEQ ID NO: 131 - protein, 21 aa, Artificial Sequence
  Anaplasma antigenic peptide
IEAGYEKFKTDGIRESGTKEC

SEQ ID NO: 132 - protein, 21 aa, Artificial Sequence
  Anaplasma antigenic peptide
IEVGYENFKTDGIRESGTKEC

SEQ ID NO: 133 - protein, 21 aa, Artificial Sequence
  Anaplasma antigenic peptide
IEVGYEQFKTDGIRESGTKEC

SEQ ID NO: 134 - protein, 21 aa, Artificial Sequence
  Anaplasma antigenic peptide
IEAGYENFKTDGIRESGTKEC

SEQ ID NO: 135 - protein, 21 aa, Artificial Sequence
  Anaplasma antigenic peptide
IEAGYEQFKTDGIRESGTKEC

SEQ ID NO: 136 - protein, 21 aa, Artificial Sequence
  Anaplasma antigenic peptide
IELGYEKFKTNGIRESGTKEC

SEQ ID NO: 137 - protein, 21 aa, Artificial Sequence
  Anaplasma antigenic peptide
IELGYENFKTNGIRESGTKEC

SEQ ID NO: 138 - protein, 21 aa, Artificial Sequence
  Anaplasma antigenic peptide
IELGYEQFKTNGIRESGTKEC

SEQ ID NO: 139 - protein, 21 aa, Artificial Sequence
  Anaplasma antigenic peptide
IEVGYEKFKTNGIRESGTKEC

SEQ ID NO: 140 - protein, 21 aa, Artificial Sequence
  Anaplasma antigenic peptide
IEAGYEKFKTNGIRESGTKEC

SEQ ID NO: 141 - protein, 21 aa, Artificial Sequence
  Anaplasma antigenic peptide
IEVGYENFKTNGIRESGTKEC

SEQ ID NO: 142 - protein, 21 aa, Artificial Sequence
  Anaplasma antigenic peptide
IEVGYEQFKTNGIRESGTKEC

SEQ ID NO: 143 - protein, 21 aa, Artificial Sequence
  Anaplasma antigenic peptide
IEAGYENFKTNGIRESGTKEC

SEQ ID NO: 144 - protein, 21 aa, Artificial Sequence
  Anaplasma antigenic peptide
IEAGYEQFKTNGIRESGTKEC

SEQ ID NO: 145 - protein, 21 aa, Artificial Sequence
  Anaplasma antigenic peptide
IELGYEKFKTRGIRNSGTKEC

SEQ ID NO: 146 - protein, 21 aa, Artificial Sequence
  Anaplasma antigenic peptide
IELGYENFKTRGIRNSGTKEC

SEQ ID NO: 147 - protein, 21 aa, Artificial Sequence
  Anaplasma antigenic peptide
IELGYEQFKTRGIRNSGTKEC

SEQ ID NO: 148 - protein, 21 aa, Artificial Sequence
  Anaplasma antigenic peptide
IEVGYEKFKTRGIRNSGTKEC

SEQ ID NO: 149 - protein, 21 aa, Artificial Sequence
  Anaplasma antigenic peptide
IEAGYEKFKTRGIRNSGTKEC

SEQ ID NO: 150 - protein, 21 aa, Artificial Sequence
  Anaplasma antigenic peptide
IEVGYENFKTRGIRNSGTKEC

SEQ ID NO: 151 - protein, 21 aa, Artificial Sequence
  Anaplasma antigenic peptide
IEVGYEQFKTRGIRNSGTKEC

SEQ ID NO: 152 - protein, 21 aa, Artificial Sequence
  Anaplasma antigenic peptide
IEAGYENFKTRGIRNSGTKEC

SEQ ID NO: 153 - protein, 21 aa, Artificial Sequence
  Anaplasma antigenic peptide
IEAGYEQFKTRGIRNSGTKEC

SEQ ID NO: 154 - protein, 21 aa, Artificial Sequence
  Anaplasma antigenic peptide
IELGYEKFKTDGIRNSGTKEC

SEQ ID NO: 155 - protein, 21 aa, Artificial Sequence
  Anaplasma antigenic peptide
IELGYENFKTDGIRNSGTKEC

SEQ ID NO: 156 - protein, 21 aa, Artificial Sequence
  Anaplasma antigenic peptide
IELGYEQFKTDGIRNSGTKEC

SEQ ID NO: 157 - protein, 21 aa, Artificial Sequence
  Anaplasma antigenic peptide
IEVGYEKFKTDGIRNSGTKEC

SEQ ID NO: 158 - protein, 21 aa, Artificial Sequence
  Anaplasma antigenic peptide
IEAGYEKFKTDGIRNSGTKEC

SEQ ID NO: 159 - protein, 21 aa, Artificial Sequence
  Anaplasma antigenic peptide
IEVGYENFKTDGIRNSGTKEC

SEQ ID NO: 160 - protein, 21 aa, Artificial Sequence
  Anaplasma antigenic peptide
IEVGYEQFKTDGIRNSGTKEC

SEQ ID NO: 161 - protein, 21 aa, Artificial Sequence
  Anaplasma antigenic peptide
IEAGYENFKTDGIRNSGTKEC

SEQ ID NO: 162 - protein, 21 aa, Artificial Sequence
  Anaplasma antigenic peptide
IEAGYEQFKTDGIRNSGTKEC

SEQ ID NO: 163 - protein, 21 aa, Artificial Sequence
  Anaplasma antigenic peptide
IELGYEKFKTNGIRNSGTKEC

SEQ ID NO: 164 - protein, 21 aa, Artificial Sequence
  Anaplasma antigenic peptide
IELGYENFKTNGIRNSGTKEC

SEQ ID NO: 165 - protein, 21 aa, Artificial Sequence
  Anaplasma antigenic peptide
IELGYEQFKTNGIRNSGTKEC

SEQ ID NO: 166 - protein, 21 aa, Artificial Sequence
  Anaplasma antigenic peptide
IEVGYEKFKTNGIRNSGTKEC

SEQ ID NO: 167 - protein, 21 aa, Artificial Sequence
  Anaplasma antigenic peptide
IEAGYEKFKTNGIRNSGTKEC

SEQ ID NO: 168 - protein, 21 aa, Artificial Sequence
  Anaplasma antigenic peptide
IEVGYENFKTNGIRNSGTKEC

SEQ ID NO: 169 - protein, 21 aa, Artificial Sequence
  Anaplasma antigenic peptide
IEVGYEQFKTNGIRNSGTKEC

SEQ ID NO: 170 - protein, 21 aa, Artificial Sequence
  Anaplasma antigenic peptide
IEAGYENFKTNGIRNSGTKEC

SEQ ID NO: 171 - protein, 21 aa, Artificial Sequence
  Anaplasma antigenic peptide
IEAGYEQFKTNGIRNSGTKEC

SEQ ID NO: 172 - protein, 21 aa, Artificial Sequence
  Anaplasma antigenic peptide
IELGYEKFKTRGIRQSGTKEC

SEQ ID NO: 173 - protein, 21 aa, Artificial Sequence
  Anaplasma antigenic peptide
IELGYENFKTRGIRQSGTKEC

SEQ ID NO: 174 - protein, 21 aa, Artificial Sequence
  Anaplasma antigenic peptide
IELGYEQFKTRGIRQSGTKEC

SEQ ID NO: 175 - protein, 21 aa, Artificial Sequence
  Anaplasma antigenic peptide
IEVGYEKFKTRGIRQSGTKEC

SEQ ID NO: 176 - protein, 21 aa, Artificial Sequence
  Anaplasma antigenic peptide
IEAGYEKFKTRGIRQSGTKEC

SEQ ID NO: 177 - protein, 21 aa, Artificial Sequence
  Anaplasma antigenic peptide
IEVGYENFKTRGIRQSGTKEC

SEQ ID NO: 178 - protein, 21 aa, Artificial Sequence
  Anaplasma antigenic peptide
IEVGYEQFKTRGIRQSGTKEC

SEQ ID NO: 179 - protein, 21 aa, Artificial Sequence
  Anaplasma antigenic peptide
IEAGYENFKTRGIRQSGTKEC

SEQ ID NO: 180 - protein, 21 aa, Artificial Sequence
  Anaplasma antigenic peptide
IEAGYEQFKTRGIRQSGTKEC

SEQ ID NO: 181 - protein, 21 aa, Artificial Sequence
  Anaplasma antigenic peptide
IELGYEKFKTDGIRQSGTKEC

SEQ ID NO: 182 - protein, 21 aa, Artificial Sequence
  Anaplasma antigenic peptide
IELGYENFKTDGIRQSGTKEC

SEQ ID NO: 183 - protein, 21 aa, Artificial Sequence
  Anaplasma antigenic peptide
IELGYEQFKTDGIRQSGTKEC

SEQ ID NO: 184 - protein, 21 aa, Artificial Sequence
  Anaplasma antigenic peptide
IEVGYEKFKTDGIRQSGTKEC

SEQ ID NO: 185 - protein, 21 aa, Artificial Sequence
  Anaplasma antigenic peptide
IEAGYEKFKTDGIRQSGTKEC

SEQ ID NO: 186 - protein, 21 aa, Artificial Sequence
  Anaplasma antigenic peptide
IEVGYENFKTDGIRQSGTKEC

SEQ ID NO: 187 - protein, 21 aa, Artificial Sequence
  Anaplasma antigenic peptide
IEVGYEQFKTDGIRQSGTKEC

SEQ ID NO: 188 - protein, 21 aa, Artificial Sequence
  Anaplasma antigenic peptide
IEAGYENFKTDGIRQSGTKEC

SEQ ID NO: 189 - protein, 21 aa, Artificial Sequence
  Anaplasma antigenic peptide
IEAGYEQFKTDGIRQSGTKEC

SEQ ID NO: 190 - protein, 21 aa, Artificial Sequence
  Anaplasma antigenic peptide
IELGYEKFKTNGIRQSGTKEC

SEQ ID NO: 191 - protein, 21 aa, Artificial Sequence
  Anaplasma antigenic peptide
IELGYENFKTNGIRQSGTKEC

SEQ ID NO: 192 - protein, 21 aa, Artificial Sequence
  Anaplasma antigenic peptide
IELGYEQFKTNGIRQSGTKEC

SEQ ID NO: 193 - protein, 21 aa, Artificial Sequence
  Anaplasma antigenic peptide
IEVGYEKFKTNGIRQSGTKEC

SEQ ID NO: 194 - protein, 21 aa, Artificial Sequence
  Anaplasma antigenic peptide
IEAGYEKFKTNGIRQSGTKEC

SEQ ID NO: 195 - protein, 21 aa, Artificial Sequence
  Anaplasma antigenic peptide
IEVGYENFKTNGIRQSGTKEC

SEQ ID NO: 196 - protein, 21 aa, Artificial Sequence
  Anaplasma antigenic peptide
IEVGYEQFKTNGIRQSGTKEC

SEQ ID NO: 197 - protein, 21 aa, Artificial Sequence
  Anaplasma antigenic peptide
IEAGYENFKTNGIRQSGTKEC

SEQ ID NO: 198 - protein, 21 aa, Artificial Sequence
  Anaplasma antigenic peptide
IEAGYEQFKTNGIRQSGTKEC

SEQ ID NO: 199 - protein, 67 aa, Artificial Sequence
  Anaplasma antigenic peptide
ETKVVYGYLKEGRTVKLDSHRFDWQTPEPKLGFKDGGGGGKDGTKVEFKADKFEWNSPDFRIIFKQC

SEQ ID NO: 200 - protein, 67 aa, Artificial Sequence
  Anaplasma antigenic peptide
ETKVVYIYLKEGRTVKLDSHRFDWQTPEPKLGFKDGGGGGKDGTKVEFKADKFEWNSPDFRIIFKQC

SEQ ID NO: 201 - protein, 67 aa, Artificial Sequence
  Anaplasma antigenic peptide
ETKVVYHYLKEGRTVKLDSHRFDWQTPEPKLGFKDGGGGGKDGTKVEFKADKFEWNSPDFRIIFKQC

SEQ ID NO: 202 - protein, 67 aa, Artificial Sequence
  Anaplasma antigenic peptide
ETKVAYGYLKEGRTVKLDSHRFDWQTPEPKLGFKDGGGGGKDGTKVEFKADKFEWNSPDFRIIFKQC

SEQ ID NO: 203 - protein, 67 aa, Artificial Sequence
  Anaplasma antigenic peptide
ETKVAYIYLKEGRTVKLDSHRFDWQTPEPKLGFKDGGGGGKDGTKVEFKADKFEWNSPDFRIIFKQC

SEQ ID NO: 204 - protein, 67 aa, Artificial Sequence
  Anaplasma antigenic peptide
ETKVAYHYLKEGRTVKLDSHRFDWQTPEPKLGFKDGGGGGKDGTKVEFKADKFEWNSPDFRIIFKQC

SEQ ID NO: 205 - protein, 67 aa, Artificial Sequence
  Anaplasma antigenic peptide
ETKVVYGYLKNGRTVKLDSHRFDWQTPEPKLGFKDGGGGGKDGTKVEFKADKFEWNSPDFRIIFKQC

SEQ ID NO: 206 - protein, 67 aa, Artificial Sequence
  Anaplasma antigenic peptide
ETKVVYIYLKNGRTVKLDSHRFDWQTPEPKLGFKDGGGGGKDGTKVEFKADKFEWNSPDFRIIFKQC

SEQ ID NO: 207 - protein, 67 aa, Artificial Sequence
  Anaplasma antigenic peptide
ETKVVYHYLKNGRTVKLDSHRFDWQTPEPKLGFKDGGGGGKDGTKVEFKADKFEWNSPDFRIIFKQC

SEQ ID NO: 208 - protein, 67 aa, Artificial Sequence
  Anaplasma antigenic peptide
ETKVAYGYLKNGRTVKLDSHRFDWQTPEPKLGFKDGGGGGKDGTKVEFKADKFEWNSPDFRIIFKQC

SEQ ID NO: 209 - protein, 67 aa, Artificial Sequence
  Anaplasma antigenic peptide
ETKVAYIYLKNGRTVKLDSHRFDWQTPEPKLGFKDGGGGGKDGTKVEFKADKFEWNSPDFRIIFKQC

SEQ ID NO: 210 - protein, 67 aa, Artificial Sequence
  Anaplasma antigenic peptide
ETKVAYHYLKNGRTVKLDSHRFDWQTPEPKLGFKDGGGGGKDGTKVEFKADKFEWNSPDFRIIFKQC

SEQ ID NO: 211 - protein, 67 aa, Artificial Sequence
  Anaplasma antigenic peptide
ETKVVYGYLKQGRTVKLDSHRFDWQTPEPKLGFKDGGGGGKDGTKVEFKADKFEWNSPDFRIIFKQC

SEQ ID NO: 212 - protein, 67 aa, Artificial Sequence
  Anaplasma antigenic peptide
ETKVVYIYLKQGRTVKLDSHRFDWQTPEPKLGFKDGGGGGKDGTKVEFKADKFEWNSPDFRIIFKQC

SEQ ID NO: 213 - protein, 67 aa, Artificial Sequence
  Anaplasma antigenic peptide
ETKVVYHYLKQGRTVKLDSHRFDWQTPEPKLGFKDGGGGGKDGTKVEFKADKFEWNSPDFRIIFKQC

SEQ ID NO: 214 - protein, 67 aa, Artificial Sequence
  Anaplasma antigenic peptide
ETKVAYGYLKQGRTVKLDSHRFDWQTPEPKLGFKDGGGGGKDGTKVEFKADKFEWNSPDFRIIFKQC

SEQ ID NO: 215 - protein, 67 aa, Artificial Sequence
  Anaplasma antigenic peptide
ETKVAYIYLKQGRTVKLDSHRFDWQTPEPKLGFKDGGGGGKDGTKVEFKADKFEWNSPDFRIIFKQC

SEQ ID NO: 216 - protein, 67 aa, Artificial Sequence
  Anaplasma antigenic peptide
ETKVAYHYLKQGRTVKLDSHRFDWQTPEPKLGFKDGGGGGKDGTKVEFKADKFEWNSPDFRIIFKQC

SEQ ID NO: 217 - protein, 67 aa, Artificial Sequence
  Anaplasma antigenic peptide
ETKVVYGYLKEGRTVKLNSHRFDWQTPEPKLGFKDGGGGGKDGTKVEFKADKFEWNSPDFRIIFKQC

SEQ ID NO: 218 - protein, 67 aa, Artificial Sequence
  Anaplasma antigenic peptide
ETKVVYIYLKEGRTVKLNSHRFDWQTPEPKLGFKDGGGGGKDGTKVEFKADKFEWNSPDFRIIFKQC

SEQ ID NO: 219 - protein, 67 aa, Artificial Sequence
  Anaplasma antigenic peptide
ETKVVYHYLKEGRTVKLNSHRFDWQTPEPKLGFKDGGGGGKDGTKVEFKADKFEWNSPDFRIIFKQC

SEQ ID NO: 220 - protein, 67 aa, Artificial Sequence
  Anaplasma antigenic peptide
ETKVAYGYLKEGRTVKLNSHRFDWQTPEPKLGFKDGGGGGKDGTKVEFKADKFEWNSPDFRIIFKQC

SEQ ID NO: 221 - protein, 67 aa, Artificial Sequence
  Anaplasma antigenic peptide
ETKVAYIYLKEGRTVKLNSHRFDWQTPEPKLGFKDGGGGGKDGTKVEFKADKFEWNSPDFRIIFKQC

SEQ ID NO: 222 - protein, 67 aa, Artificial Sequence
  Anaplasma antigenic peptide
ETKVAYHYLKEGRTVKLNSHRFDWQTPEPKLGFKDGGGGGKDGTKVEFKADKFEWNSPDFRIIFKQC

SEQ ID NO: 223 - protein, 67 aa, Artificial Sequence
  Anaplasma antigenic peptide
ETKVVYGYLKNGRTVKLNSHRFDWQTPEPKLGFKDGGGGGKDGTKVEFKADKFEWNSPDFRIIFKQC

SEQ ID NO: 224 - protein, 67 aa, Artificial Sequence
  Anaplasma antigenic peptide
ETKVVYIYLKNGRTVKLNSHRFDWQTPEPKLGFKDGGGGGKDGTKVEFKADKFEWNSPDFRIIFKQC

SEQ ID NO: 225 - protein, 67 aa, Artificial Sequence
  Anaplasma antigenic peptide
ETKVVYHYLKNGRTVKLNSHRFDWQTPEPKLGFKDGGGGGKDGTKVEFKADKFEWNSPDFRIIFKQC

SEQ ID NO: 226 - protein, 67 aa, Artificial Sequence
  Anaplasma antigenic peptide
ETKVAYGYLKNGRTVKLNSHRFDWQTPEPKLGFKDGGGGGKDGTKVEFKADKFEWNSPDFRIIFKQC

SEQ ID NO: 227 - protein, 67 aa, Artificial Sequence
  Anaplasma antigenic peptide
ETKVAYIYLKNGRTVKLNSHRFDWQTPEPKLGFKDGGGGGKDGTKVEFKADKFEWNSPDFRIIFKQC

SEQ ID NO: 228 - protein, 67 aa, Artificial Sequence
  Anaplasma antigenic peptide
ETKVAYHYLKNGRTVKLNSHRFDWQTPEPKLGFKDGGGGGKDGTKVEFKADKFEWNSPDFRIIFKQC

SEQ ID NO: 229 - protein, 67 aa, Artificial Sequence
  Anaplasma antigenic peptide
ETKVVYGYLKQGRTVKLNSHRFDWQTPEPKLGFKDGGGGGKDGTKVEFKADKFEWNSPDFRIIFKQC

SEQ ID NO: 230 - protein, 67 aa, Artificial Sequence
  Anaplasma antigenic peptide
ETKVVYIYLKQGRTVKLNSHRFDWQTPEPKLGFKDGGGGGKDGTKVEFKADKFEWNSPDFRIIFKQC

SEQ ID NO: 231 - protein, 67 aa, Artificial Sequence
  Anaplasma antigenic peptide
ETKVVYHYLKQGRTVKLNSHRFDWQTPEPKLGFKDGGGGGKDGTKVEFKADKFEWNSPDFRIIFKQC

SEQ ID NO: 232 - protein, 67 aa, Artificial Sequence
  Anaplasma antigenic peptide
ETKVAYGYLKQGRTVKLNSHRFDWQTPEPKLGFKDGGGGGKDGTKVEFKADKFEWNSPDFRIIFKQC

SEQ ID NO: 233 - protein, 67 aa, Artificial Sequence
  Anaplasma antigenic peptide
ETKVAYIYLKQGRTVKLNSHRFDWQTPEPKLGFKDGGGGGKDGTKVEFKADKFEWNSPDFRIIFKQC

SEQ ID NO: 234 - protein, 67 aa, Artificial Sequence
  Anaplasma antigenic peptide
ETKVAYHYLKQGRTVKLNSHRFDWQTPEPKLGFKDGGGGGKDGTKVEFKADKFEWNSPDFRIIFKQC

SEQ ID NO: 235 - protein, 67 aa, Artificial Sequence
  Anaplasma antigenic peptide
ETKVVYGYLKEGRTVKLDSHDFDWQTPEPKLGFKDGGGGGKDGTKVEFKADKFEWNSPDFRIIFKQC

SEQ ID NO: 236 - protein, 67 aa, Artificial Sequence
  Anaplasma antigenic peptide
ETKVVYIYLKEGRTVKLDSHDFDWQTPEPKLGFKDGGGGGKDGTKVEFKADKFEWNSPDFRIIFKQC

SEQ ID NO: 237 - protein, 67 aa, Artificial Sequence
  Anaplasma antigenic peptide
ETKVVYHYLKEGRTVKLDSHDFDWQTPEPKLGFKDGGGGGKDGTKVEFKADKFEWNSPDFRIIFKQC

SEQ ID NO: 238 - protein, 67 aa, Artificial Sequence
  Anaplasma antigenic peptide
ETKVAYGYLKEGRTVKLDSHDFDWQTPEPKLGFKDGGGGGKDGTKVEFKADKFEWNSPDFRIIFKQC

SEQ ID NO: 239 - protein, 67 aa, Artificial Sequence
  Anaplasma antigenic peptide
ETKVAYIYLKEGRTVKLDSHDFDWQTPEPKLGFKDGGGGGKDGTKVEFKADKFEWNSPDFRIIFKQC

SEQ ID NO: 240 - protein, 67 aa, Artificial Sequence
  Anaplasma antigenic peptide
ETKVAYHYLKEGRTVKLDSHDFDWQTPEPKLGFKDGGGGGKDGTKVEFKADKFEWNSPDFRIIFKQC

SEQ ID NO: 241 - protein, 67 aa, Artificial Sequence
  Anaplasma antigenic peptide
ETKVVYGYLKNGRTVKLDSHDFDWQTPEPKLGFKDGGGGGKDGTKVEFKADKFEWNSPDFRIIFKQC

SEQ ID NO: 242 - protein, 67 aa, Artificial Sequence
  Anaplasma antigenic peptide
ETKVVYIYLKNGRTVKLDSHDFDWQTPEPKLGFKDGGGGGKDGTKVEFKADKFEWNSPDFRIIFKQC

SEQ ID NO: 243 - protein, 67 aa, Artificial Sequence
  Anaplasma antigenic peptide
ETKVVYHYLKNGRTVKLDSHDFDWQTPEPKLGFKDGGGGGKDGTKVEFKADKFEWNSPDFRIIFKQC

SEQ ID NO: 244 - protein, 67 aa, Artificial Sequence
  Anaplasma antigenic peptide
ETKVAYGYLKNGRTVKLDSHDFDWQTPEPKLGFKDGGGGGKDGTKVEFKADKFEWNSPDFRIIFKQC

SEQ ID NO: 245 - protein, 67 aa, Artificial Sequence
  Anaplasma antigenic peptide
ETKVAYIYLKNGRTVKLDSHDFDWQTPEPKLGFKDGGGGGKDGTKVEFKADKFEWNSPDFRIIFKQC

SEQ ID NO: 246 - protein, 67 aa, Artificial Sequence
  Anaplasma antigenic peptide
ETKVAYHYLKNGRTVKLDSHDFDWQTPEPKLGFKDGGGGGKDGTKVEFKADKFEWNSPDFRIIFKQC

SEQ ID NO: 247 - protein, 67 aa, Artificial Sequence
  Anaplasma antigenic peptide
ETKVVYGYLKQGRTVKLDSHDFDWQTPEPKLGFKDGGGGGKDGTKVEFKADKFEWNSPDFRIIFKQC

SEQ ID NO: 248 - protein, 67 aa, Artificial Sequence
  Anaplasma antigenic peptide
ETKVVYIYLKQGRTVKLDSHDFDWQTPEPKLGFKDGGGGGKDGTKVEFKADKFEWNSPDFRIIFKQC

SEQ ID NO: 249 - protein, 67 aa, Artificial Sequence
  Anaplasma antigenic peptide
ETKVVYHYLKQGRTVKLDSHDFDWQTPEPKLGFKDGGGGGKDGTKVEFKADKFEWNSPDFRIIFKQC

SEQ ID NO: 250 - protein, 67 aa, Artificial Sequence
  Anaplasma antigenic peptide
ETKVAYGYLKQGRTVKLDSHDFDWQTPEPKLGFKDGGGGGKDGTKVEFKADKFEWNSPDFRIIFKQC

SEQ ID NO: 251 - protein, 67 aa, Artificial Sequence
  Anaplasma antigenic peptide
ETKVAYIYLKQGRTVKLDSHDFDWQTPEPKLGFKDGGGGGKDGTKVEFKADKFEWNSPDFRIIFKQC

SEQ ID NO: 252 - protein, 67 aa, Artificial Sequence
  Anaplasma antigenic peptide
ETKVAYHYLKQGRTVKLDSHDFDWQTPEPKLGFKDGGGGGKDGTKVEFKADKFEWNSPDFRIIFKQC

SEQ ID NO: 253 - protein, 67 aa, Artificial Sequence
  Anaplasma antigenic peptide
ETKVVYGYLKEGRTVKLNSHDFDWQTPEPKLGFKDGGGGGKDGTKVEFKADKFEWNSPDFRIIFKQC

SEQ ID NO: 254 - protein, 67 aa, Artificial Sequence
  Anaplasma antigenic peptide
ETKVVYIYLKEGRTVKLNSHDFDWQTPEPKLGFKDGGGGGKDGTKVEFKADKFEWNSPDFRIIFKQC

SEQ ID NO: 255 - protein, 67 aa, Artificial Sequence
  Anaplasma antigenic peptide
ETKVVYHYLKEGRTVKLNSHDFDWQTPEPKLGFKDGGGGGKDGTKVEFKADKFEWNSPDFRIIFKQC

SEQ ID NO: 256 - protein, 67 aa, Artificial Sequence
  Anaplasma antigenic peptide
ETKVAYGYLKEGRTVKLNSHDFDWQTPEPKLGFKDGGGGGKDGTKVEFKADKFEWNSPDFRIIFKQC

SEQ ID NO: 257 - protein, 67 aa, Artificial Sequence
  Anaplasma antigenic peptide
ETKVAYIYLKEGRTVKLNSHDFDWQTPEPKLGFKDGGGGGKDGTKVEFKADKFEWNSPDFRIIFKQC

SEQ ID NO: 258 - protein, 67 aa, Artificial Sequence
  Anaplasma antigenic peptide
ETKVAYHYLKEGRTVKLNSHDFDWQTPEPKLGFKDGGGGGKDGTKVEFKADKFEWNSPDFRIIFKQC

SEQ ID NO: 259 - protein, 67 aa, Artificial Sequence
  Anaplasma antigenic peptide
ETKVVYGYLKNGRTVKLNSHDFDWQTPEPKLGFKDGGGGGKDGTKVEFKADKFEWNSPDFRIIFKQC

SEQ ID NO: 260 - protein, 67 aa, Artificial Sequence
  Anaplasma antigenic peptide
ETKVVYIYLKNGRTVKLNSHDFDWQTPEPKLGFKDGGGGGKDGTKVEFKADKFEWNSPDFRIIFKQC

SEQ ID NO: 261 - protein, 67 aa, Artificial Sequence
  Anaplasma antigenic peptide
ETKVVYHYLKNGRTVKLNSHDFDWQTPEPKLGFKDGGGGGKDGTKVEFKADKFEWNSPDFRIIFKQC

SEQ ID NO: 262 - protein, 67 aa, Artificial Sequence
  Anaplasma antigenic peptide
ETKVAYGYLKNGRTVKLNSHDFDWQTPEPKLGFKDGGGGGKDGTKVEFKADKFEWNSPDFRIIFKQC

SEQ ID NO: 263 - protein, 67 aa, Artificial Sequence
  Anaplasma antigenic peptide
ETKVAYIYLKNGRTVKLNSHDFDWQTPEPKLGFKDGGGGGKDGTKVEFKADKFEWNSPDFRIIFKQC

SEQ ID NO: 264 - protein, 67 aa, Artificial Sequence
  Anaplasma antigenic peptide
ETKVAYHYLKNGRTVKLNSHDFDWQTPEPKLGFKDGGGGGKDGTKVEFKADKFEWNSPDFRIIFKQC

SEQ ID NO: 265 - protein, 67 aa, Artificial Sequence
  Anaplasma antigenic peptide
ETKVVYGYLKQGRTVKLNSHDFDWQTPEPKLGFKDGGGGGKDGTKVEFKADKFEWNSPDFRIIFKQC

SEQ ID NO: 266 - protein, 67 aa, Artificial Sequence
  Anaplasma antigenic peptide
ETKVVYIYLKQGRTVKLNSHDFDWQTPEPKLGFKDGGGGGKDGTKVEFKADKFEWNSPDFRIIFKQC

SEQ ID NO: 267 - protein, 67 aa, Artificial Sequence
  Anaplasma antigenic peptide
ETKVVYHYLKQGRTVKLNSHDFDWQTPEPKLGFKDGGGGGKDGTKVEFKADKFEWNSPDFRIIFKQC

SEQ ID NO: 268 - protein, 67 aa, Artificial Sequence
  Anaplasma antigenic peptide
ETKVAYGYLKQGRTVKLNSHDFDWQTPEPKLGFKDGGGGGKDGTKVEFKADKFEWNSPDFRIIFKQC

SEQ ID NO: 269 - protein, 67 aa, Artificial Sequence
  Anaplasma antigenic peptide
ETKVAYIYLKQGRTVKLNSHDFDWQTPEPKLGFKDGGGGGKDGTKVEFKADKFEWNSPDFRIIFKQC

SEQ ID NO: 270 - protein, 67 aa, Artificial Sequence
  Anaplasma antigenic peptide
ETKVAYHYLKQGRTVKLNSHDFDWQTPEPKLGFKDGGGGGKDGTKVEFKADKFEWNSPDFRIIFKQC

SEQ ID NO: 271 - protein, 67 aa, Artificial Sequence
  Anaplasma antigenic peptide
ETKVVYGYLKEGRTVKLDSHNFDWQTPEPKLGFKDGGGGGKDGTKVEFKADKFEWNSPDFRIIFKQC

SEQ ID NO: 272 - protein, 67 aa, Artificial Sequence
  Anaplasma antigenic peptide
ETKVVYIYLKEGRTVKLDSHNFDWQTPEPKLGFKDGGGGGKDGTKVEFKADKFEWNSPDFRIIFKQC

SEQ ID NO: 273 - protein, 67 aa, Artificial Sequence
  Anaplasma antigenic peptide
ETKVVYHYLKEGRTVKLDSHNFDWQTPEPKLGFKDGGGGGKDGTKVEFKADKFEWNSPDFRIIFKQC

SEQ ID NO: 274 - protein, 67 aa, Artificial Sequence
  Anaplasma antigenic peptide
ETKVAYGYLKEGRTVKLDSHNFDWQTPEPKLGFKDGGGGGKDGTKVEFKADKFEWNSPDFRIIFKQC

SEQ ID NO: 275 - protein, 67 aa, Artificial Sequence
  Anaplasma antigenic peptide
ETKVAYIYLKEGRTVKLDSHNFDWQTPEPKLGFKDGGGGGKDGTKVEFKADKFEWNSPDFRIIFKQC

SEQ ID NO: 276 - protein, 67 aa, Artificial Sequence
  Anaplasma antigenic peptide
ETKVAYHYLKEGRTVKLDSHNFDWQTPEPKLGFKDGGGGGKDGTKVEFKADKFEWNSPDFRIIFKQC

SEQ ID NO: 277 - protein, 67 aa, Artificial Sequence
  Anaplasma antigenic peptide
ETKVVYGYLKNGRTVKLDSHNFDWQTPEPKLGFKDGGGGGKDGTKVEFKADKFEWNSPDFRIIFKQC

SEQ ID NO: 278 - protein, 67 aa, Artificial Sequence
  Anaplasma antigenic peptide
ETKVVYIYLKNGRTVKLDSHNFDWQTPEPKLGFKDGGGGGKDGTKVEFKADKFEWNSPDFRIIFKQC

SEQ ID NO: 279 - protein, 67 aa, Artificial Sequence
  Anaplasma antigenic peptide
ETKVVYHYLKNGRTVKLDSHNFDWQTPEPKLGFKDGGGGGKDGTKVEFKADKFEWNSPDFRIIFKQC

SEQ ID NO: 280 - protein, 67 aa, Artificial Sequence
  Anaplasma antigenic peptide
ETKVAYGYLKNGRTVKLDSHNFDWQTPEPKLGFKDGGGGGKDGTKVEFKADKFEWNSPDFRIIFKQC

SEQ ID NO: 281 - protein, 67 aa, Artificial Sequence
  Anaplasma antigenic peptide
ETKVAYIYLKNGRTVKLDSHNFDWQTPEPKLGFKDGGGGGKDGTKVEFKADKFEWNSPDFRIIFKQC

SEQ ID NO: 282 - protein, 67 aa, Artificial Sequence
  Anaplasma antigenic peptide
ETKVAYHYLKNGRTVKLDSHNFDWQTPEPKLGFKDGGGGGKDGTKVEFKADKFEWNSPDFRIIFKQC

SEQ ID NO: 283 - protein, 67 aa, Artificial Sequence
  Anaplasma antigenic peptide
ETKVVYGYLKQGRTVKLDSHNFDWQTPEPKLGFKDGGGGGKDGTKVEFKADKFEWNSPDFRIIFKQC

SEQ ID NO: 284 - protein, 67 aa, Artificial Sequence
  Anaplasma antigenic peptide
ETKVVYIYLKQGRTVKLDSHNFDWQTPEPKLGFKDGGGGGKDGTKVEFKADKFEWNSPDFRIIFKQC

SEQ ID NO: 285 - protein, 67 aa, Artificial Sequence
  Anaplasma antigenic peptide
ETKVVYHYLKQGRTVKLDSHNFDWQTPEPKLGFKDGGGGGKDGTKVEFKADKFEWNSPDFRIIFKQC

SEQ ID NO: 286 - protein, 67 aa, Artificial Sequence
  Anaplasma antigenic peptide
ETKVAYGYLKQGRTVKLDSHNFDWQTPEPKLGFKDGGGGGKDGTKVEFKADKFEWNSPDFRIIFKQC

SEQ ID NO: 287 - protein, 67 aa, Artificial Sequence
  Anaplasma antigenic peptide
ETKVAYIYLKQGRTVKLDSHNFDWQTPEPKLGFKDGGGGGKDGTKVEFKADKFEWNSPDFRIIFKQC

SEQ ID NO: 288 - protein, 67 aa, Artificial Sequence
  Anaplasma antigenic peptide
ETKVAYHYLKQGRTVKLDSHNFDWQTPEPKLGFKDGGGGGKDGTKVEFKADKFEWNSPDFRIIFKQC

SEQ ID NO: 289 - protein, 67 aa, Artificial Sequence
  Anaplasma antigenic peptide
ETKVVYGYLKEGRTVKLNSHNFDWQTPEPKLGFKDGGGGGKDGTKVEFKADKFEWNSPDFRIIFKQC

SEQ ID NO: 290 - protein, 67 aa, Artificial Sequence
  Anaplasma antigenic peptide
ETKVVYIYLKEGRTVKLNSHNFDWQTPEPKLGFKDGGGGGKDGTKVEFKADKFEWNSPDFRIIFKQC

SEQ ID NO: 291 - protein, 67 aa, Artificial Sequence
  Anaplasma antigenic peptide
ETKVVYHYLKEGRTVKLNSHNFDWQTPEPKLGFKDGGGGGKDGTKVEFKADKFEWNSPDFRIIFKQC

SEQ ID NO: 292 - protein, 67 aa, Artificial Sequence
  Anaplasma antigenic peptide
ETKVAYGYLKEGRTVKLNSHNFDWQTPEPKLGFKDGGGGGKDGTKVEFKADKFEWNSPDFRIIFKQC

SEQ ID NO: 293 - protein, 67 aa, Artificial Sequence
  Anaplasma antigenic peptide
ETKVAYIYLKEGRTVKLNSHNFDWQTPEPKLGFKDGGGGGKDGTKVEFKADKFEWNSPDFRIIFKQC

SEQ ID NO: 294 - protein, 67 aa, Artificial Sequence
  Anaplasma antigenic peptide
ETKVAYHYLKEGRTVKLNSHNFDWQTPEPKLGFKDGGGGGKDGTKVEFKADKFEWNSPDFRIIFKQC

SEQ ID NO: 295 - protein, 67 aa, Artificial Sequence
  Anaplasma antigenic peptide
ETKVVYGYLKNGRTVKLNSHNFDWQTPEPKLGFKDGGGGGKDGTKVEFKADKFEWNSPDFRIIFKQC

SEQ ID NO: 296 - protein, 67 aa, Artificial Sequence
  Anaplasma antigenic peptide
ETKVVYIYLKNGRTVKLNSHNFDWQTPEPKLGFKDGGGGGKDGTKVEFKADKFEWNSPDFRIIFKQC

SEQ ID NO: 297 - protein, 67 aa, Artificial Sequence
  Anaplasma antigenic peptide
ETKVVYHYLKNGRTVKLNSHNFDWQTPEPKLGFKDGGGGGKDGTKVEFKADKFEWNSPDFRIIFKQC

SEQ ID NO: 298 - protein, 67 aa, Artificial Sequence
  Anaplasma antigenic peptide
ETKVAYGYLKNGRTVKLNSHNFDWQTPEPKLGFKDGGGGGKDGTKVEFKADKFEWNSPDFRIIFKQC

SEQ ID NO: 299 - protein, 67 aa, Artificial Sequence
  Anaplasma antigenic peptide
ETKVAYIYLKNGRTVKLNSHNFDWQTPEPKLGFKDGGGGGKDGTKVEFKADKFEWNSPDFRIIFKQC

SEQ ID NO: 300 - protein, 67 aa, Artificial Sequence
  Anaplasma antigenic peptide
ETKVAYHYLKNGRTVKLNSHNFDWQTPEPKLGFKDGGGGGKDGTKVEFKADKFEWNSPDFRIIFKQC

SEQ ID NO: 301 - protein, 67 aa, Artificial Sequence
  Anaplasma antigenic peptide
ETKVVYGYLKQGRTVKLNSHNFDWQTPEPKLGFKDGGGGGKDGTKVEFKADKFEWNSPDFRIIFKQC

SEQ ID NO: 302 - protein, 67 aa, Artificial Sequence
  Anaplasma antigenic peptide
ETKVVYIYLKQGRTVKLNSHNFDWQTPEPKLGFKDGGGGGKDGTKVEFKADKFEWNSPDFRIIFKQC

SEQ ID NO: 303 - protein, 67 aa, Artificial Sequence
  Anaplasma antigenic peptide
ETKVVYHYLKQGRTVKLNSHNFDWQTPEPKLGFKDGGGGGKDGTKVEFKADKFEWNSPDFRIIFKQC

SEQ ID NO: 304 - protein, 67 aa, Artificial Sequence
  Anaplasma antigenic peptide
ETKVAYGYLKQGRTVKLNSHNFDWQTPEPKLGFKDGGGGGKDGTKVEFKADKFEWNSPDFRIIFKQC

SEQ ID NO: 305 - protein, 67 aa, Artificial Sequence
  Anaplasma antigenic peptide
ETKVAYIYLKQGRTVKLNSHNFDWQTPEPKLGFKDGGGGGKDGTKVEFKADKFEWNSPDFRIIFKQC

SEQ ID NO: 306 - protein, 67 aa, Artificial Sequence
  Anaplasma antigenic peptide
ETKVAYHYLKQGRTVKLNSHNFDWQTPEPKLGFKDGGGGGKDGTKVEFKADKFEWNSPDFRIIFKQC

SEQ ID NO: 307 - protein, 67 aa, Artificial Sequence
  Anaplasma antigenic peptide
ETKVVYGYLKEGRTVKLDSHRFDWQTPEPKLGFKDGGGGGKDGTKVEFKADKFEWNSPDFRIIFKDC

SEQ ID NO: 308 - protein, 67 aa, Artificial Sequence
  Anaplasma antigenic peptide
ETKVVYIYLKEGRTVKLDSHRFDWQTPEPKLGFKDGGGGGKDGTKVEFKADKFEWNSPDFRIIFKDC

SEQ ID NO: 309 - protein, 67 aa, Artificial Sequence
  Anaplasma antigenic peptide
ETKVVYHYLKEGRTVKLDSHRFDWQTPEPKLGFKDGGGGGKDGTKVEFKADKFEWNSPDFRIIFKDC

SEQ ID NO: 310 - protein, 67 aa, Artificial Sequence
  Anaplasma antigenic peptide
ETKVAYGYLKEGRTVKLDSHRFDWQTPEPKLGFKDGGGGGKDGTKVEFKADKFEWNSPDFRIIFKDC

SEQ ID NO: 311 - protein, 67 aa, Artificial Sequence
  Anaplasma antigenic peptide
ETKVAYIYLKEGRTVKLDSHRFDWQTPEPKLGFKDGGGGGKDGTKVEFKADKFEWNSPDFRIIFKDC

SEQ ID NO: 312 - protein, 67 aa, Artificial Sequence
  Anaplasma antigenic peptide
ETKVAYHYLKEGRTVKLDSHRFDWQTPEPKLGFKDGGGGGKDGTKVEFKADKFEWNSPDFRIIFKDC

SEQ ID NO: 313 - protein, 67 aa, Artificial Sequence
  Anaplasma antigenic peptide
ETKVVYGYLKNGRTVKLDSHRFDWQTPEPKLGFKDGGGGGKDGTKVEFKADKFEWNSPDFRIIFKDC

SEQ ID NO: 314 - protein, 67 aa, Artificial Sequence
  Anaplasma antigenic peptide
ETKVVYIYLKNGRTVKLDSHRFDWQTPEPKLGFKDGGGGGKDGTKVEFKADKFEWNSPDFRIIFKDC

SEQ ID NO: 315 - protein, 67 aa, Artificial Sequence
  Anaplasma antigenic peptide
ETKVVYHYLKNGRTVKLDSHRFDWQTPEPKLGFKDGGGGGKDGTKVEFKADKFEWNSPDFRIIFKDC

SEQ ID NO: 316 - protein, 67 aa, Artificial Sequence
  Anaplasma antigenic peptide
ETKVAYGYLKNGRTVKLDSHRFDWQTPEPKLGFKDGGGGGKDGTKVEFKADKFEWNSPDFRIIFKDC

SEQ ID NO: 317 - protein, 67 aa, Artificial Sequence
  Anaplasma antigenic peptide
ETKVVYGYLKEGRTVKLDSHRFDWQTPEPKLGFKDGGGGGKDGTKVEFKADKFEWNSPDFRIVFKDC

SEQ ID NO: 318 - protein, 67 aa, Artificial Sequence
  Anaplasma antigenic peptide
ETKVVYIYLKEGRTVKLDSHRFDWQTPEPKLGFKDGGGGGKDGTKVEFKADKFEWNSPDFRIVFKDC

SEQ ID NO: 319 - protein, 67 aa, Artificial Sequence
  Anaplasma antigenic peptide
ETKVVYHYLKEGRTVKLDSHRFDWQTPEPKLGFKDGGGGGKDGTKVEFKADKFEWNSPDFRIVFKDC

SEQ ID NO: 320 - protein, 67 aa, Artificial Sequence
  Anaplasma antigenic peptide
ETKVAYGYLKEGRTVKLDSHRFDWQTPEPKLGFKDGGGGGKDGTKVEFKADKFEWNSPDFRIVFKDC

SEQ ID NO: 321 - protein, 67 aa, Artificial Sequence
  Anaplasma antigenic peptide
ETKVAYIYLKEGRTVKLDSHRFDWQTPEPKLGFKDGGGGGKDGTKVEFKADKFEWNSPDFRIVFKDC

SEQ ID NO: 322 - protein, 67 aa, Artificial Sequence
  Anaplasma antigenic peptide
ETKVAYHYLKEGRTVKLDSHRFDWQTPEPKLGFKDGGGGGKDGTKVEFKADKFEWNSPDFRIVFKDC

SEQ ID NO: 323 - protein, 67 aa, Artificial Sequence
  Anaplasma antigenic peptide
ETKVVYGYLKNGRTVKLDSHRFDWQTPEPKLGFKDGGGGGKDGTKVEFKADKFEWNSPDFRIVFKDC

SEQ ID NO: 324 - protein, 67 aa, Artificial Sequence
  Anaplasma antigenic peptide
ETKVVYIYLKNGRTVKLDSHRFDWQTPEPKLGFKDGGGGGKDGTKVEFKADKFEWNSPDFRIVFKDC

SEQ ID NO: 325 - protein, 67 aa, Artificial Sequence
  Anaplasma antigenic peptide
ETKVVYHYLKNGRTVKLDSHRFDWQTPEPKLGFKDGGGGGKDGTKVEFKADKFEWNSPDFRIVFKDC

SEQ ID NO: 326 - protein, 67 aa, Artificial Sequence
  Anaplasma antigenic peptide
ETKVAYGYLKNGRTVKLDSHRFDWQTPEPKLGFKDGGGGGKDGTKVEFKADKFEWNSPDFRIVFKDC

SEQ ID NO: 327 - protein, 67 aa, Artificial Sequence
  Anaplasma antigenic peptide
ETKVVYGYLKEGRTVKLDSHRFDWQTPEPKLGFKDGGGGGKDGTKVEFKADKFEWNSPDWRIVFKDC

SEQ ID NO: 328 - protein, 67 aa, Artificial Sequence
  Anaplasma antigenic peptide
ETKVVYIYLKEGRTVKLDSHRFDWQTPEPKLGFKDGGGGGKDGTKVEFKADKFEWNSPDWRIVFKDC

SEQ ID NO: 329 - protein, 67 aa, Artificial Sequence
  Anaplasma antigenic peptide
ETKVVYHYLKEGRTVKLDSHRFDWQTPEPKLGFKDGGGGGKDGTKVEFKADKFEWNSPDWRIVFKDC

SEQ ID NO: 330 - protein, 67 aa, Artificial Sequence
  Anaplasma antigenic peptide
ETKVAYGYLKEGRTVKLDSHRFDWQTPEPKLGFKDGGGGGKDGTKVEFKADKFEWNSPDWRIVFKDC

SEQ ID NO: 331 - protein, 67 aa, Artificial Sequence
  Anaplasma antigenic peptide
ETKVAYIYLKEGRTVKLDSHRFDWQTPEPKLGFKDGGGGGKDGTKVEFKADKFEWNSPDWRIVFKDC

SEQ ID NO: 332 - protein, 67 aa, Artificial Sequence
  Anaplasma antigenic peptide
ETKVAYHYLKEGRTVKLDSHRFDWQTPEPKLGFKDGGGGGKDGTKVEFKADKFEWNSPDWRIVFKDC

SEQ ID NO: 333 - protein, 67 aa, Artificial Sequence
  Anaplasma antigenic peptide
ETKVVYGYLKNGRTVKLDSHRFDWQTPEPKLGFKDGGGGGKDGTKVEFKADKFEWNSPDWRIVFKDC

SEQ ID NO: 334 - protein, 67 aa, Artificial Sequence
  Anaplasma antigenic peptide
ETKVVYIYLKNGRTVKLDSHRFDWQTPEPKLGFKDGGGGGKDGTKVEFKADKFEWNSPDWRIVFKDC

SEQ ID NO: 335 - protein, 67 aa, Artificial Sequence
  Anaplasma antigenic peptide
ETKVVYHYLKNGRTVKLDSHRFDWQTPEPKLGFKDGGGGGKDGTKVEFKADKFEWNSPDWRIVFKDC

SEQ ID NO: 336 - protein, 67 aa, Artificial Sequence
  Anaplasma antigenic peptide
ETKVAYGYLKNGRTVKLDSHRFDWQTPEPKLGFKDGGGGGKDGTKVEFKADKFEWNSPDWRIVFKDC

SEQ ID NO: 337 - protein, 67 aa, Artificial Sequence
  Anaplasma antigenic peptide
ETKVVYGYLKEGRTVKLDSHRFDWQTPEPKLGFKDGGGGGKDGTKVEFKADKFEWNQPDWRIVFKDC

SEQ ID NO: 338 - protein, 67 aa, Artificial Sequence
  Anaplasma antigenic peptide
ETKVVYIYLKEGRTVKLDSHRFDWQTPEPKLGFKDGGGGGKDGTKVEFKADKFEWNQPDWRIVFKDC

SEQ ID NO: 339 - protein, 67 aa, Artificial Sequence
  Anaplasma antigenic peptide
ETKVVYHYLKEGRTVKLDSHRFDWQTPEPKLGFKDGGGGGKDGTKVEFKADKFEWNQPDWRIVFKDC

SEQ ID NO: 340 - protein, 67 aa, Artificial Sequence
  Anaplasma antigenic peptide
ETKVAYGYLKEGRTVKLDSHRFDWQTPEPKLGFKDGGGGGKDGTKVEFKADKFEWNQPDWRIVFKDC

SEQ ID NO: 341 - protein, 67 aa, Artificial Sequence
  Anaplasma antigenic peptide
ETKVAYIYLKEGRTVKLDSHRFDWQTPEPKLGFKDGGGGGKDGTKVEFKADKFEWNQPDWRIVFKDC

SEQ ID NO: 342 - protein, 67 aa, Artificial Sequence
  Anaplasma antigenic peptide
ETKVAYHYLKEGRTVKLDSHRFDWQTPEPKLGFKDGGGGGKDGTKVEFKADKFEWNQPDWRIVFKDC

SEQ ID NO: 343 - protein, 67 aa, Artificial Sequence
  Anaplasma antigenic peptide
ETKVVYGYLKNGRTVKLDSHRFDWQTPEPKLGFKDGGGGGKDGTKVEFKADKFEWNQPDWRIVFKDC

SEQ ID NO: 344 - protein, 67 aa, Artificial Sequence
  Anaplasma antigenic peptide
ETKVVYIYLKNGRTVKLDSHRFDWQTPEPKLGFKDGGGGGKDGTKVEFKADKFEWNQPDWRIVFKDC

SEQ ID NO: 345 - protein, 67 aa, Artificial Sequence
  Anaplasma antigenic peptide
ETKVVYHYLKNGRTVKLDSHRFDWQTPEPKLGFKDGGGGGKDGTKVEFKADKFEWNQPDWRIVFKDC

SEQ ID NO: 346 - protein, 67 aa, Artificial Sequence
  Anaplasma antigenic peptide
ETKVAYGYLKNGRTVKLDSHRFDWQTPEPKLGFKDGGGGGKDGTKVEFKADKFEWNQPDWRIVFKDC

SEQ ID NO: 347 - protein, 67 aa, Artificial Sequence
  Anaplasma antigenic peptide
ETKVVYGYLKEGRTVKLDSHRFDWQTPEPKLGFKDGGGGGKDGTKVEFKADKFQWNQPDWRIVFKDC

SEQ ID NO: 348 - protein, 67 aa, Artificial Sequence
  Anaplasma antigenic peptide
ETKVVYIYLKEGRTVKLDSHRFDWQTPEPKLGFKDGGGGGKDGTKVEFKADKFQWNQPDWRIVFKDC

SEQ ID NO: 349 - protein, 67 aa, Artificial Sequence
  Anaplasma antigenic peptide
ETKVVYGYLKEGRTVKLDSHRFDWQTPEPKLGFKDGGGGGKDGTKVEFKANKFQWNQPDWRIVFKDC

SEQ ID NO: 350 - protein, 67 aa, Artificial Sequence
  Anaplasma antigenic peptide
ETKVVYIYLKEGRTVKLDSHRFDWQTPEPKLGFKDGGGGGKDGTKVEFKANKFQWNQPDWRIVFKDC

SEQ ID NO: 351 - protein, 27 aa, Artificial Sequence
  Anaplasma antigenic peptide
CKDGTKVEFKADKFEWNSPDFRIIFKQ

SEQ ID NO: 352 - protein, 27 aa, Artificial Sequence
  Anaplasma antigenic peptide
CKDGTKVEVKADKFEWNSPDFRIIFKQ

SEQ ID NO: 353 - protein, 27 aa, Artificial Sequence
  Anaplasma antigenic peptide
CKDGTQVEFKADKFEWNSPDFRIIFKQ

SEQ ID NO: 354 - protein, 27 aa, Artificial Sequence
  Anaplasma antigenic peptide
CKDGTQVEVKADKFEWNSPDFRIIFKQ

SEQ ID NO: 355 - protein, 27 aa, Artificial Sequence
  Anaplasma antigenic peptide
CKDGTKVEFKANKFEWNSPDFRIIFKQ

SEQ ID NO: 356 - protein, 27 aa, Artificial Sequence
  Anaplasma antigenic peptide
CKDGTKVEVKANKFEWNSPDFRIIFKQ

SEQ ID NO: 357 - protein, 27 aa, Artificial Sequence
  Anaplasma antigenic peptide
CKDGTQVEFKANKFEWNSPDFRIIFKQ

SEQ ID NO: 358 - protein, 27 aa, Artificial Sequence
  Anaplasma antigenic peptide
CKDGTQVEVKANKFEWNSPDFRIIFKQ

SEQ ID NO: 359 - protein, 27 aa, Artificial Sequence
  Anaplasma antigenic peptide
CKDGTKVEFKADKFQWNSPDFRIIFKQ

SEQ ID NO: 360 - protein, 27 aa, Artificial Sequence
  Anaplasma antigenic peptide
CKDGTKVEVKADKFQWNSPDFRIIFKQ

SEQ ID NO: 361 - protein, 27 aa, Artificial Sequence
  Anaplasma antigenic peptide
CKDGTQVEFKADKFQWNSPDFRIIFKQ

SEQ ID NO: 362 - protein, 27 aa, Artificial Sequence
  Anaplasma antigenic peptide
CKDGTQVEVKADKFQWNSPDFRIIFKQ

SEQ ID NO: 363 - protein, 27 aa, Artificial Sequence
  Anaplasma antigenic peptide
CKDGTKVEFKANKFQWNSPDFRIIFKQ

SEQ ID NO: 364 - protein, 27 aa, Artificial Sequence
  Anaplasma antigenic peptide
CKDGTKVEVKANKFQWNSPDFRIIFKQ

SEQ ID NO: 365 - protein, 27 aa, Artificial Sequence
  Anaplasma antigenic peptide
CKDGTQVEFKANKFQWNSPDFRIIFKQ

SEQ ID NO: 366 - protein, 27 aa, Artificial Sequence
  Anaplasma antigenic peptide
CKDGTQVEVKANKFQWNSPDFRIIFKQ

SEQ ID NO: 367 - protein, 27 aa, Artificial Sequence
  Anaplasma antigenic peptide
CKDGTKVEFKADKFQWNQPDFRIIFKQ

SEQ ID NO: 368 - protein, 27 aa, Artificial Sequence
  Anaplasma antigenic peptide
CKDGTKVEVKADKFQWNQPDFRIIFKQ

SEQ ID NO: 369 - protein, 27 aa, Artificial Sequence
  Anaplasma antigenic peptide
CKDGTQVEFKADKFQWNQPDFRIIFKQ

SEQ ID NO: 370 - protein, 27 aa, Artificial Sequence
  Anaplasma antigenic peptide
CKDGTQVEVKADKFQWNQPDFRIIFKQ

SEQ ID NO: 371 - protein, 27 aa, Artificial Sequence
  Anaplasma antigenic peptide
CKDGTKVEFKANKFQWNQPDFRIIFKQ

SEQ ID NO: 372 - protein, 27 aa, Artificial Sequence
  Anaplasma antigenic peptide
CKDGTKVEVKANKFQWNQPDFRIIFKQ

SEQ ID NO: 373 - protein, 27 aa, Artificial Sequence
  Anaplasma antigenic peptide
CKDGTQVEFKANKFQWNQPDFRIIFKQ

SEQ ID NO: 374 - protein, 27 aa, Artificial Sequence
  Anaplasma antigenic peptide
CKDGTQVEVKANKFQWNQPDFRIIFKQ

SEQ ID NO: 375 - protein, 27 aa, Artificial Sequence
  Anaplasma antigenic peptide
CKDGTKVEFKADKFQWNQPDWRIIFKQ

SEQ ID NO: 376 - protein, 27 aa, Artificial Sequence
  Anaplasma antigenic peptide
CKDGTKVEVKADKFQWNQPDWRIIFKQ

SEQ ID NO: 377 - protein, 27 aa, Artificial Sequence
  Anaplasma antigenic peptide
CKDGTQVEFKADKFQWNQPDWRIIFKQ

SEQ ID NO: 378 - protein, 27 aa, Artificial Sequence
  Anaplasma antigenic peptide
CKDGTQVEVKADKFQWNQPDWRIIFKQ

SEQ ID NO: 379 - protein, 27 aa, Artificial Sequence
  Anaplasma antigenic peptide
CKDGTKVEFKANKFQWNQPDWRIIFKQ

SEQ ID NO: 380 - protein, 27 aa, Artificial Sequence
  Anaplasma antigenic peptide
CKDGTKVEVKANKFQWNQPDWRIIFKQ

SEQ ID NO: 381 - protein, 27 aa, Artificial Sequence
  Anaplasma antigenic peptide
CKDGTQVEFKANKFQWNQPDWRIIFKQ

SEQ ID NO: 382 - protein, 27 aa, Artificial Sequence
  Anaplasma antigenic peptide
CKDGTQVEVKANKFQWNQPDWRIIFKQ

SEQ ID NO: 383 - protein, 27 aa, Artificial Sequence
  Anaplasma antigenic peptide
CKDGTKVEFKADKFQWNQPDWRIVFKQ

SEQ ID NO: 384 - protein, 27 aa, Artificial Sequence
  Anaplasma antigenic peptide
CKDGTKVEVKADKFQWNQPDWRIVFKQ

SEQ ID NO: 385 - protein, 27 aa, Artificial Sequence
  Anaplasma antigenic peptide
CKDGTQVEFKADKFQWNQPDWRIVFKQ

SEQ ID NO: 386 - protein, 27 aa, Artificial Sequence
  Anaplasma antigenic peptide
CKDGTQVEVKADKFQWNQPDWRIVFKQ

SEQ ID NO: 387 - protein, 27 aa, Artificial Sequence
  Anaplasma antigenic peptide
CKDGTKVEFKANKFQWNQPDWRIVFKQ

SEQ ID NO: 388 - protein, 27 aa, Artificial Sequence
  Anaplasma antigenic peptide
CKDGTKVEVKANKFQWNQPDWRIVFKQ

SEQ ID NO: 389 - protein, 27 aa, Artificial Sequence
  Anaplasma antigenic peptide
CKDGTQVEFKANKFQWNQPDWRIVFKQ

SEQ ID NO: 390 - protein, 27 aa, Artificial Sequence
  Anaplasma antigenic peptide
CKDGTQVEVKANKFQWNQPDWRIVFKQ

SEQ ID NO: 391 - protein, 27 aa, Artificial Sequence
  Anaplasma antigenic peptide
CKDGTKVEFKADKFQWNQPDWRIVFKD

SEQ ID NO: 392 - protein, 27 aa, Artificial Sequence
  Anaplasma antigenic peptide
CKDGTKVEVKADKFQWNQPDWRIVFKD

SEQ ID NO: 393 - protein, 27 aa, Artificial Sequence
  Anaplasma antigenic peptide
CKDGTQVEFKADKFQWNQPDWRIVFKD

SEQ ID NO: 394 - protein, 27 aa, Artificial Sequence
  Anaplasma antigenic peptide
CKDGTQVEVKADKFQWNQPDWRIVFKD

SEQ ID NO: 395 - protein, 27 aa, Artificial Sequence
  Anaplasma antigenic peptide
CKDGTKVEFKANKFQWNQPDWRIVFKD

SEQ ID NO: 396 - protein, 27 aa, Artificial Sequence
  Anaplasma antigenic peptide
CKDGTKVEVKANKFQWNQPDWRIVFKD

SEQ ID NO: 397 - protein, 27 aa, Artificial Sequence
  Anaplasma antigenic peptide
CKDGTQVEFKANKFQWNQPDWRIVFKD

SEQ ID NO: 398 - protein, 27 aa, Artificial Sequence
  Anaplasma antigenic peptide
CKDGTQVEVKANKFQWNQPDWRIVFKD

SEQ ID NO: 399 - protein, 40 aa, Artificial Sequence
  Anaplasma antigenic peptide
CIGGKSPARSTEERVAGDLDHKEVDSDKKHDAEKTEEKRH

SEQ ID NO: 400 - protein, 40 aa, Artificial Sequence
  Anaplasma antigenic peptide
CIGGKSPARYTEERVAGDLDHKEVDSDKKHDAEKTEEKRH

SEQ ID NO: 401 - protein, 40 aa, Artificial Sequence
  Anaplasma antigenic peptide
CVGGKSPARSTEERVAGDLDHKEVDSDKKHDAEKTEEKRH

SEQ ID NO: 402 - protein, 40 aa, Artificial Sequence
  Anaplasma antigenic peptide
CVGGKSPARYTEERVAGDLDHKEVDSDKKHDAEKTEEKRH

SEQ ID NO: 403 - protein, 40 aa, Artificial Sequence
  Anaplasma antigenic peptide
CIGGKSPARSTEERVAGDLDHKNVDSDKKHDAEKTEEKRH

SEQ ID NO: 404 - protein, 40 aa, Artificial Sequence
  Anaplasma antigenic peptide
CIGGKSPARYTEERVAGDLDHKNVDSDKKHDAEKTEEKRH

SEQ ID NO: 405 - protein, 40 aa, Artificial Sequence
  Anaplasma antigenic peptide
CVGGKSPARSTEERVAGDLDHKNVDSDKKHDAEKTEEKRH

SEQ ID NO: 406 - protein, 40 aa, Artificial Sequence
  Anaplasma antigenic peptide
CVGGKSPARYTEERVAGDLDHKNVDSDKKHDAEKTEEKRH

SEQ ID NO: 407 - protein, 27 aa, Artificial Sequence
  Anaplasma antigenic peptide
CKDGSRVEFKAERFNWQSPNPKIKYRN

SEQ ID NO: 408 - protein, 27 aa, Artificial Sequence
  Anaplasma antigenic peptide
CKDGSRVEYKAERFNWQSPNPKIKYRN

SEQ ID NO: 409 - protein, 27 aa, Artificial Sequence
  Anaplasma antigenic peptide
CKDGQRVEFKAERFNWQSPNPKIKYRN

SEQ ID NO: 410 - protein, 27 aa, Artificial Sequence
  Anaplasma antigenic peptide
CKDGQRVEYKAERFNWQSPNPKIKYRN

SEQ ID NO: 411 - protein, 27 aa, Artificial Sequence
  Anaplasma antigenic peptide
CKDGSRVEFKAEHFNWQSPNPKIKYRN

SEQ ID NO: 412 - protein, 27 aa, Artificial Sequence
  Anaplasma antigenic peptide
CKDGSRVEYKAEHFNWQSPNPKIKYRN

SEQ ID NO: 413 - protein, 27 aa, Artificial Sequence
  Anaplasma antigenic peptide
CKDGQRVEFKAEHFNWQSPNPKIKYRN

SEQ ID NO: 414 - protein, 27 aa, Artificial Sequence
  Anaplasma antigenic peptide
CKDGQRVEYKAEHFNWQSPNPKIKYRN

SEQ ID NO: 415 - protein, 27 aa, Artificial Sequence
  Anaplasma antigenic peptide
CKDGSRVEFKAERFNYQSPNPKIKYRN

SEQ ID NO: 416 - protein, 27 aa, Artificial Sequence
  Anaplasma antigenic peptide
CKDGSRVEYKAERFNYQSPNPKIKYRN

SEQ ID NO: 417 - protein, 27 aa, Artificial Sequence
  Anaplasma antigenic peptide
CKDGQRVEFKAERFNYQSPNPKIKYRN

SEQ ID NO: 418 - protein, 27 aa, Artificial Sequence
  Anaplasma antigenic peptide
CKDGQRVEYKAERFNYQSPNPKIKYRN

SEQ ID NO: 419 - protein, 27 aa, Artificial Sequence
  Anaplasma antigenic peptide
CKDGSRVEFKAEHFNYQSPNPKIKYRN

SEQ ID NO: 420 - protein, 27 aa, Artificial Sequence
  Anaplasma antigenic peptide
CKDGSRVEYKAEHFNYQSPNPKIKYRN

SEQ ID NO: 421 - protein, 27 aa, Artificial Sequence
  Anaplasma antigenic peptide
CKDGQRVEFKAEHFNYQSPNPKIKYRN

SEQ ID NO: 422 - protein, 27 aa, Artificial Sequence
  Anaplasma antigenic peptide
CKDGQRVEYKAEHFNYQSPNPKIKYRN

SEQ ID NO: 423 - protein, 27 aa, Artificial Sequence
  Anaplasma antigenic peptide
CKDGSRVEFKAERFNWQQPNPKIKYRN

SEQ ID NO: 424 - protein, 27 aa, Artificial Sequence
  Anaplasma antigenic peptide
CKDGSRVEYKAERFNWQQPNPKIKYRN

SEQ ID NO: 425 - protein, 27 aa, Artificial Sequence
  Anaplasma antigenic peptide
CKDGQRVEFKAERFNWQQPNPKIKYRN

SEQ ID NO: 426 - protein, 27 aa, Artificial Sequence
  Anaplasma antigenic peptide
CKDGQRVEYKAERFNWQQPNPKIKYRN

SEQ ID NO: 427 - protein, 27 aa, Artificial Sequence
  Anaplasma antigenic peptide
CKDGSRVEFKAEHFNWQQPNPKIKYRN

SEQ ID NO: 428 - protein, 27 aa, Artificial Sequence
  Anaplasma antigenic peptide
CKDGSRVEYKAEHFNWQQPNPKIKYRN

SEQ ID NO: 429 - protein, 27 aa, Artificial Sequence
  Anaplasma antigenic peptide
CKDGQRVEFKAEHFNWQQPNPKIKYRN

SEQ ID NO: 430 - protein, 27 aa, Artificial Sequence
  Anaplasma antigenic peptide
CKDGQRVEYKAEHFNWQQPNPKIKYRN

SEQ ID NO: 431 - protein, 27 aa, Artificial Sequence
  Anaplasma antigenic peptide
CKDGSRVEFKAERFNYQQPNPKIKYRN

SEQ ID NO: 432 - protein, 27 aa, Artificial Sequence
  Anaplasma antigenic peptide
CKDGSRVEYKAERFNYQQPNPKIKYRN

SEQ ID NO: 433 - protein, 27 aa, Artificial Sequence
  Anaplasma antigenic peptide
CKDGQRVEFKAERFNYQQPNPKIKYRN

SEQ ID NO: 434 - protein, 27 aa, Artificial Sequence
  Anaplasma antigenic peptide
CKDGQRVEYKAERFNYQQPNPKIKYRN

SEQ ID NO: 435 - protein, 27 aa, Artificial Sequence
  Anaplasma antigenic peptide
CKDGSRVEFKAEHFNYQQPNPKIKYRN

SEQ ID NO: 436 - protein, 27 aa, Artificial Sequence
  Anaplasma antigenic peptide
CKDGSRVEYKAEHFNYQQPNPKIKYRN

SEQ ID NO: 437 - protein, 27 aa, Artificial Sequence
  Anaplasma antigenic peptide
CKDGQRVEFKAEHFNYQQPNPKIKYRN

SEQ ID NO: 438 - protein, 27 aa, Artificial Sequence
  Anaplasma antigenic peptide
CKDGQRVEYKAEHFNYQQPNPKIKYRN

SEQ ID NO: 439 - protein, 27 aa, Artificial Sequence
  Anaplasma antigenic peptide
CKDGQRVEFKAEHFNWQQPNPHIKYRN

SEQ ID NO: 440 - protein, 27 aa, Artificial Sequence
  Anaplasma antigenic peptide
CKDGQRVEYKAEHFNWQQPNPHIKYRN

SEQ ID NO: 441 - protein, 27 aa, Artificial Sequence
  Anaplasma antigenic peptide
CKDGSRVEFKAERFNYQQPNPHIKYRN

SEQ ID NO: 442 - protein, 27 aa, Artificial Sequence
  Anaplasma antigenic peptide
CKDGSRVEYKAERFNYQQPNPHIKYRN

SEQ ID NO: 443 - protein, 27 aa, Artificial Sequence
  Anaplasma antigenic peptide
CKDGQRVEFKAERFNYQQPNPHIKYRN

SEQ ID NO: 444 - protein, 27 aa, Artificial Sequence
  Anaplasma antigenic peptide
CKDGQRVEYKAERFNYQQPNPHIKYRN

SEQ ID NO: 445 - protein, 27 aa, Artificial Sequence
  Anaplasma antigenic peptide
CKDGSRVEFKAEHFNYQQPNPHIKYRN

SEQ ID NO: 446 - protein, 27 aa, Artificial Sequence
  Anaplasma antigenic peptide
CKDGSRVEYKAEHFNYQQPNPHIKYRN

SEQ ID NO: 447 - protein, 27 aa, Artificial Sequence
  Anaplasma antigenic peptide
CKDGQRVEFKAEHFNYQQPNPHIKYRN

SEQ ID NO: 448 - protein, 27 aa, Artificial Sequence
  Anaplasma antigenic peptide
CKDGQRVEYKAEHFNYQQPNPHIKYRN

SEQ ID NO: 449 - protein, 27 aa, Artificial Sequence
  Anaplasma antigenic peptide
CKDGQRVEFKAEHFNWQQPNPHIKYRD

SEQ ID NO: 450 - protein, 27 aa, Artificial Sequence
  Anaplasma antigenic peptide
CKDGQRVEYKAEHFNWQQPNPHIKYRD

SEQ ID NO: 451 - protein, 27 aa, Artificial Sequence
  Anaplasma antigenic peptide
CKDGSRVEFKAERFNYQQPNPHIKYRD

SEQ ID NO: 452 - protein, 27 aa, Artificial Sequence
  Anaplasma antigenic peptide
CKDGSRVEYKAERFNYQQPNPHIKYRD

SEQ ID NO: 453 - protein, 27 aa, Artificial Sequence
  Anaplasma antigenic peptide
CKDGQRVEFKAERFNYQQPNPHIKYRD

SEQ ID NO: 454 - protein, 27 aa, Artificial Sequence
  Anaplasma antigenic peptide
CKDGQRVEYKAERFNYQQPNPHIKYRD

SEQ ID NO: 455 - protein, 27 aa, Artificial Sequence
  Anaplasma antigenic peptide
CKDGSRVEFKAEHFNYQQPNPHIKYRD

SEQ ID NO: 456 - protein, 27 aa, Artificial Sequence
  Anaplasma antigenic peptide
CKDGSRVEYKAEHFNYQQPNPHIKYRD

SEQ ID NO: 457 - protein, 27 aa, Artificial Sequence
  Anaplasma antigenic peptide
CKDGQRVEFKAEHFNYQQPNPHIKYRD

SEQ ID NO: 458 - protein, 27 aa, Artificial Sequence
  Anaplasma antigenic peptide
CKDGQRVEYKAEHFNYQQPNPHIKYRD

SEQ ID NO: 459 - protein, 31 aa, Artificial Sequence
  Anaplasma antigenic peptide
CGKILNLVSVANEKKPPEAPAADEAAGPATH

SEQ ID NO: 460 - protein, 31 aa, Artificial Sequence
  Anaplasma antigenic peptide
CGKILNLVSVLNEKKPPEAPAADEAAGPATH

SEQ ID NO: 461 - protein, 31 aa, Artificial Sequence
  Anaplasma antigenic peptide
CGKILNLVSLANEKKPPEAPAADEAAGPATH

SEQ ID NO: 462 - protein, 31 aa, Artificial Sequence
  Anaplasma antigenic peptide
CGKILNLVSLLNEKKPPEAPAADEAAGPATH

SEQ ID NO: 463 - protein, 31 aa, Artificial Sequence
  Anaplasma antigenic peptide
CGKILNLVSIANEKKPPEAPAADEAAGPATH

SEQ ID NO: 464 - protein, 31 aa, Artificial Sequence
  Anaplasma antigenic peptide
CGKILNLVSILNEKKPPEAPAADEAAGPATH

SEQ ID NO: 465 - protein, 36 aa, Artificial Sequence
  Anaplasma antigenic peptide
ETKVVYGYLKEGRTVKLDSHRFDWQTPEPKLGFKDC

SEQ ID NO: 466 - protein, 36 aa, Artificial Sequence
  Anaplasma antigenic peptide
ETKVVYIYLKEGRTVKLDSHRFDWQTPEPKLGFKDC

SEQ ID NO: 467 - protein, 36 aa, Artificial Sequence
  Anaplasma antigenic peptide
ETKVVYHYLKEGRTVKLDSHRFDWQTPEPKLGFKDC

SEQ ID NO: 468 - protein, 36 aa, Artificial Sequence
  Anaplasma antigenic peptide
ETKVAYGYLKEGRTVKLDSHRFDWQTPEPKLGFKDC

SEQ ID NO: 469 - protein, 36 aa, Artificial Sequence
  Anaplasma antigenic peptide
ETKVAYIYLKEGRTVKLDSHRFDWQTPEPKLGFKDC

SEQ ID NO: 470 - protein, 36 aa, Artificial Sequence
  Anaplasma antigenic peptide
ETKVAYHYLKEGRTVKLDSHRFDWQTPEPKLGFKDC

SEQ ID NO: 471 - protein, 36 aa, Artificial Sequence
  Anaplasma antigenic peptide
ETKVVYGYLKNGRTVKLDSHRFDWQTPEPKLGFKDC

SEQ ID NO: 472 - protein, 36 aa, Artificial Sequence
  Anaplasma antigenic peptide
ETKVVYIYLKNGRTVKLDSHRFDWQTPEPKLGFKDC

SEQ ID NO: 473 - protein, 36 aa, Artificial Sequence
  Anaplasma antigenic peptide
ETKVVYHYLKNGRTVKLDSHRFDWQTPEPKLGFKDC

SEQ ID NO: 474 - protein, 36 aa, Artificial Sequence
  Anaplasma antigenic peptide
ETKVAYGYLKNGRTVKLDSHRFDWQTPEPKLGFKDC

SEQ ID NO: 475 - protein, 36 aa, Artificial Sequence
  Anaplasma antigenic peptide
ETKVAYIYLKNGRTVKLDSHRFDWQTPEPKLGFKDC

SEQ ID NO: 476 - protein, 36 aa, Artificial Sequence
  Anaplasma antigenic peptide
ETKVAYHYLKNGRTVKLDSHRFDWQTPEPKLGFKDC

SEQ ID NO: 477 - protein, 36 aa, Artificial Sequence
  Anaplasma antigenic peptide
ETKVVYGYLKQGRTVKLDSHRFDWQTPEPKLGFKDC

SEQ ID NO: 478 - protein, 36 aa, Artificial Sequence
  Anaplasma antigenic peptide
ETKVVYIYLKQGRTVKLDSHRFDWQTPEPKLGFKDC

SEQ ID NO: 479 - protein, 36 aa, Artificial Sequence
  Anaplasma antigenic peptide
ETKVVYHYLKQGRTVKLDSHRFDWQTPEPKLGFKDC

SEQ ID NO: 480 - protein, 36 aa, Artificial Sequence
  Anaplasma antigenic peptide
ETKVAYGYLKQGRTVKLDSHRFDWQTPEPKLGFKDC

SEQ ID NO: 481 - protein, 36 aa, Artificial Sequence
  Anaplasma antigenic peptide
ETKVAYIYLKQGRTVKLDSHRFDWQTPEPKLGFKDC

SEQ ID NO: 482 - protein, 36 aa, Artificial Sequence
  Anaplasma antigenic peptide
ETKVAYHYLKQGRTVKLDSHRFDWQTPEPKLGFKDC

SEQ ID NO: 483 - protein, 36 aa, Artificial Sequence
  Anaplasma antigenic peptide
ETKVVYGYLKQGRTVKLDSHDFDWQTPEPKLGFKDC

SEQ ID NO: 484 - protein, 36 aa, Artificial Sequence
  Anaplasma antigenic peptide
ETKVVYIYLKQGRTVKLDSHDFDWQTPEPKLGFKDC

SEQ ID NO: 485 - protein, 36 aa, Artificial Sequence
  Anaplasma antigenic peptide
ETKVVYHYLKQGRTVKLDSHDFDWQTPEPKLGFKDC

SEQ ID NO: 486 - protein, 36 aa, Artificial Sequence
  Anaplasma antigenic peptide
ETKVAYGYLKQGRTVKLDSHDFDWQTPEPKLGFKDC

SEQ ID NO: 487 - protein, 36 aa, Artificial Sequence
  Anaplasma antigenic peptide
ETKVAYIYLKQGRTVKLDSHDFDWQTPEPKLGFKDC

SEQ ID NO: 488 - protein, 36 aa, Artificial Sequence
  Anaplasma antigenic peptide
ETKVAYHYLKQGRTVKLDSHDFDWQTPEPKLGFKDC

SEQ ID NO: 489 - protein, 36 aa, Artificial Sequence
  Anaplasma antigenic peptide
ETKVVYGYLKQGRTVKLDSHNFDWQTPEPKLGFKDC

SEQ ID NO: 490 - protein, 36 aa, Artificial Sequence
  Anaplasma antigenic peptide
ETKVVYIYLKQGRTVKLDSHNFDWQTPEPKLGFKDC

SEQ ID NO: 491 - protein, 36 aa, Artificial Sequence
  Anaplasma antigenic peptide
ETKVVYHYLKQGRTVKLDSHNFDWQTPEPKLGFKDC

SEQ ID NO: 492 - protein, 36 aa, Artificial Sequence
  Anaplasma antigenic peptide
ETKVAYGYLKQGRTVKLDSHNFDWQTPEPKLGFKDC

SEQ ID NO: 493 - protein, 36 aa, Artificial Sequence
  Anaplasma antigenic peptide
ETKVAYIYLKQGRTVKLDSHNFDWQTPEPKLGFKDC

SEQ ID NO: 494 - protein, 36 aa, Artificial Sequence
  Anaplasma antigenic peptide
ETKVAYHYLKQGRTVKLDSHNFDWQTPEPKLGFKDC

SEQ ID NO: 495 - protein, 36 aa, Artificial Sequence
  Anaplasma antigenic peptide
ETKVVYGYLKQGRTVKLDSHDFDWDTPEPKLGFKDC

SEQ ID NO: 496 - protein, 36 aa, Artificial Sequence
  Anaplasma antigenic peptide
ETKVVYIYLKQGRTVKLDSHDFDWDTPEPKLGFKDC

SEQ ID NO: 497 - protein, 36 aa, Artificial Sequence
  Anaplasma antigenic peptide
ETKVVYHYLKQGRTVKLDSHDFDWDTPEPKLGFKDC

SEQ ID NO: 498 - protein, 36 aa, Artificial Sequence
  Anaplasma antigenic peptide
ETKVAYGYLKQGRTVKLDSHDFDWDTPEPKLGFKDC

SEQ ID NO: 499 - protein, 36 aa, Artificial Sequence
  Anaplasma antigenic peptide
ETKVAYIYLKQGRTVKLDSHDFDWDTPEPKLGFKDC

SEQ ID NO: 500 - protein, 36 aa, Artificial Sequence
  Anaplasma antigenic peptide
ETKVAYHYLKQGRTVKLDSHDFDWDTPEPKLGFKDC

SEQ ID NO: 501 - protein, 36 aa, Artificial Sequence
  Anaplasma antigenic peptide
ETKVVYGYLKQGRTVKLDSHNFDWDTPEPKLGFKDC

SEQ ID NO: 502 - protein, 36 aa, Artificial Sequence
  Anaplasma antigenic peptide
ETKVVYIYLKQGRTVKLDSHNFDWDTPEPKLGFKDC

SEQ ID NO: 503 - protein, 36 aa, Artificial Sequence
  Anaplasma antigenic peptide
ETKVVYHYLKQGRTVKLDSHNFDWDTPEPKLGFKDC

SEQ ID NO: 504 - protein, 36 aa, Artificial Sequence
  Anaplasma antigenic peptide
ETKVAYGYLKQGRTVKLDSHNFDWDTPEPKLGFKDC

SEQ ID NO: 505 - protein, 36 aa, Artificial Sequence
  Anaplasma antigenic peptide
ETKVAYIYLKQGRTVKLDSHNFDWDTPEPKLGFKDC

SEQ ID NO: 506 - protein, 36 aa, Artificial Sequence
  Anaplasma antigenic peptide
ETKVAYHYLKQGRTVKLDSHNFDWDTPEPKLGFKDC

SEQ ID NO: 507 - protein, 36 aa, Artificial Sequence
  Anaplasma antigenic peptide
ETKVVYGYLKQGRTVKLDSHDFDWETPEPKLGFKDC

SEQ ID NO: 508 - protein, 36 aa, Artificial Sequence
  Anaplasma antigenic peptide
ETKVVYIYLKQGRTVKLDSHDFDWETPEPKLGFKDC

SEQ ID NO: 509 - protein, 36 aa, Artificial Sequence
  Anaplasma antigenic peptide
ETKVVYHYLKQGRTVKLDSHDFDWETPEPKLGFKDC

SEQ ID NO: 510 - protein, 36 aa, Artificial Sequence
  Anaplasma antigenic peptide
ETKVAYGYLKQGRTVKLDSHDFDWETPEPKLGFKDC

SEQ ID NO: 511 - protein, 36 aa, Artificial Sequence
  Anaplasma antigenic peptide
ETKVAYIYLKQGRTVKLDSHDFDWETPEPKLGFKDC

SEQ ID NO: 512 - protein, 36 aa, Artificial Sequence
  Anaplasma antigenic peptide
ETKVAYHYLKQGRTVKLDSHDFDWETPEPKLGFKDC

SEQ ID NO: 513 - protein, 36 aa, Artificial Sequence
  Anaplasma antigenic peptide
ETKVVYGYLKQGRTVKLDSHNFDWETPEPKLGFKDC

SEQ ID NO: 514 - protein, 36 aa, Artificial Sequence
  Anaplasma antigenic peptide
ETKVVYIYLKQGRTVKLDSHNFDWETPEPKLGFKDC

SEQ ID NO: 515 - protein, 36 aa, Artificial Sequence
  Anaplasma antigenic peptide
ETKVVYHYLKQGRTVKLDSHNFDWETPEPKLGFKDC

SEQ ID NO: 516 - protein, 36 aa, Artificial Sequence
  Anaplasma antigenic peptide
ETKVAYGYLKQGRTVKLDSHNFDWETPEPKLGFKDC

SEQ ID NO: 517 - protein, 36 aa, Artificial Sequence
  Anaplasma antigenic peptide
ETKVAYIYLKQGRTVKLDSHNFDWETPEPKLGFKDC

SEQ ID NO: 518 - protein, 36 aa, Artificial Sequence
  Anaplasma antigenic peptide
ETKVAYHYLKQGRTVKLDSHNFDWETPEPKLGFKDC

SEQ ID NO: 519 - protein, 36 aa, Artificial Sequence
  Anaplasma antigenic peptide
ETKVVYGYLKQGRTVKLDSHDFDWETPNPKLGFKDC

SEQ ID NO: 520 - protein, 36 aa, Artificial Sequence
  Anaplasma antigenic peptide
ETKVVYIYLKQGRTVKLDSHDFDWETPNPKLGFKDC

SEQ ID NO: 521 - protein, 36 aa, Artificial Sequence
  Anaplasma antigenic peptide
ETKVVYHYLKQGRTVKLDSHDFDWETPNPKLGFKDC

SEQ ID NO: 522 - protein, 36 aa, Artificial Sequence
  Anaplasma antigenic peptide
ETKVAYGYLKQGRTVKLDSHDFDWETPNPKLGFKDC

SEQ ID NO: 523 - protein, 36 aa, Artificial Sequence
  Anaplasma antigenic peptide
ETKVAYIYLKQGRTVKLDSHDFDWETPNPKLGFKDC

SEQ ID NO: 524 - protein, 36 aa, Artificial Sequence
  Anaplasma antigenic peptide
ETKVAYHYLKQGRTVKLDSHDFDWETPNPKLGFKDC

SEQ ID NO: 525 - protein, 36 aa, Artificial Sequence
  Anaplasma antigenic peptide
ETKVVYGYLKQGRTVKLDSHNFDWETPNPKLGFKDC

SEQ ID NO: 526 - protein, 36 aa, Artificial Sequence
  Anaplasma antigenic peptide
ETKVVYIYLKQGRTVKLDSHNFDWETPNPKLGFKDC

SEQ ID NO: 527 - protein, 36 aa, Artificial Sequence
  Anaplasma antigenic peptide
ETKVVYHYLKQGRTVKLDSHNFDWETPNPKLGFKDC

SEQ ID NO: 528 - protein, 36 aa, Artificial Sequence
  Anaplasma antigenic peptide
ETKVAYGYLKQGRTVKLDSHNFDWETPNPKLGFKDC

SEQ ID NO: 529 - protein, 36 aa, Artificial Sequence
  Anaplasma antigenic peptide
ETKVAYIYLKQGRTVKLDSHNFDWETPNPKLGFKDC

SEQ ID NO: 530 - protein, 36 aa, Artificial Sequence
  Anaplasma antigenic peptide
ETKVAYHYLKQGRTVKLDSHNFDWETPNPKLGFKDC

SEQ ID NO: 531 - protein, 36 aa, Artificial Sequence
  Anaplasma antigenic peptide
ETKVVYGYLKQGRTVKLDSHDFDWETPNPKVGFKDC

SEQ ID NO: 532 - protein, 36 aa, Artificial Sequence
  Anaplasma antigenic peptide
ETKVVYIYLKQGRTVKLDSHDFDWETPNPKVGFKDC

SEQ ID NO: 533 - protein, 36 aa, Artificial Sequence
  Anaplasma antigenic peptide
ETKVVYHYLKQGRTVKLDSHDFDWETPNPKVGFKDC

SEQ ID NO: 534 - protein, 36 aa, Artificial Sequence
  Anaplasma antigenic peptide
ETKVAYGYLKQGRTVKLDSHDFDWETPNPKVGFKDC

SEQ ID NO: 535 - protein, 36 aa, Artificial Sequence
  Anaplasma antigenic peptide
ETKVAYIYLKQGRTVKLDSHDFDWETPNPKVGFKDC

SEQ ID NO: 536 - protein, 36 aa, Artificial Sequence
  Anaplasma antigenic peptide
ETKVAYHYLKQGRTVKLDSHDFDWETPNPKVGFKDC

SEQ ID NO: 537 - protein, 36 aa, Artificial Sequence
  Anaplasma antigenic peptide
ETKVVYGYLKQGRTVKLDSHNFDWETPNPKVGFKDC

SEQ ID NO: 538 - protein, 36 aa, Artificial Sequence
  Anaplasma antigenic peptide
ETKVVYIYLKQGRTVKLDSHNFDWETPNPKVGFKDC

SEQ ID NO: 539 - protein, 36 aa, Artificial Sequence
  Anaplasma antigenic peptide
ETKVVYHYLKQGRTVKLDSHNFDWETPNPKVGFKDC

SEQ ID NO: 540 - protein, 36 aa, Artificial Sequence
  Anaplasma antigenic peptide
ETKVAYGYLKQGRTVKLDSHNFDWETPNPKVGFKDC

SEQ ID NO: 541 - protein, 36 aa, Artificial Sequence
  Anaplasma antigenic peptide
ETKVAYIYLKQGRTVKLDSHNFDWETPNPKVGFKDC

SEQ ID NO: 542 - protein, 36 aa, Artificial Sequence
  Anaplasma antigenic peptide
ETKVAYHYLKQGRTVKLDSHNFDWETPNPKVGFKDC

SEQ ID NO: 543 - protein, 35 aa, Artificial Sequence
  Anaplasma antigenic peptide
  MISC_FEATURE (5)..(5): Xaa is Val or Ala
  MISC_FEATURE (7)..(7): Xaa is Gly, Ile or His
  MISC_FEATURE (11)..(11): Xaa is Glu, Asn or Gln
  MISC_FEATURE (18)..(18): Xaa is Asp or Asn
  MISC_FEATURE (21)..(21): Xaa is Arg, Asp or Asn
  MISC_FEATURE (25)..(25): Xaa is Gln, Asp or Glu
  MISC_FEATURE (28)..(28): Xaa is Glu or Asn
  MISC_FEATURE (31)..(31): Xaa is Leu or Val
ETKVXYXYLKXGRTVKLXSHXFDWXTPXPKXGFKD